European Patent Specification EP 3 689 370 B1, published March 4, 2026. Title: ANTI-GDF15 ANTIBODIES. Applicant: AVEO PHARMACEUTICALS, INC. Application Divisional of EP 13 827 058.2. The sequence listing filed with the application follows.

SEQUENCE LISTING (266 sequences)

SEQ ID NO: 1 - protein, 5 aa, Artificial Sequence
  source: /note="Description of Artificial Sequence: Synthetic peptide"
DYNMD

SEQ ID NO: 2 - protein, 5 aa, Artificial Sequence
  source: /note="Description of Artificial Sequence: Synthetic peptide"
SYWIH

SEQ ID NO: 3 - protein, 7 aa, Artificial Sequence
  source: /note="Description of Artificial Sequence: Synthetic peptide"
TYGMGVT

SEQ ID NO: 4 - protein, 7 aa, Artificial Sequence
  source: /note="Description of Artificial Sequence: Synthetic peptide"
TYGMGVS

SEQ ID NO: 5 - protein, 7 aa, Artificial Sequence
  source: /note="Description of Artificial Sequence: Synthetic peptide"
TYGMGVG

SEQ ID NO: 6 - protein, 7 aa, Artificial Sequence
  source: /note="Description of Artificial Sequence: Synthetic peptide"
TSGMGVS

SEQ ID NO: 7 - protein, 17 aa, Artificial Sequence
  source: /note="Description of Artificial Sequence: Synthetic peptide"
QINPNNGGIFFNQKFKG

SEQ ID NO: 8 - protein, 17 aa, Artificial Sequence
  source: /note="Description of Artificial Sequence: Synthetic peptide"
DINPSNGRSKYNEKFKN

SEQ ID NO: 9 - protein, 16 aa, Artificial Sequence
  source: /note="Description of Artificial Sequence: Synthetic peptide"
HIYWDDDKRYNPSLKS

SEQ ID NO: 10 - protein, 17 aa, Artificial Sequence
  source: /note="Description of Artificial Sequence: Synthetic peptide"
EINPNNGGTFYNQKFKG

SEQ ID NO: 11 - protein, 16 aa, Artificial Sequence
  source: /note="Description of Artificial Sequence: Synthetic peptide"
DIWWDDDKYYNPSLKS

SEQ ID NO: 12 - protein, 16 aa, Artificial Sequence
  source: /note="Description of Artificial Sequence: Synthetic peptide"
HNDWDDDKRYKSSLKS

SEQ ID NO: 13 - protein, 17 aa, Artificial Sequence
  source: /note="Description of Artificial Sequence: Synthetic peptide"
QINPNNGGIFFNQKFQG

SEQ ID NO: 14 - protein, 16 aa, Artificial Sequence
  source: /note="Description of Artificial Sequence: Synthetic peptide"
HIYWDDDKRYNPSLKT

SEQ ID NO: 15 - protein, 11 aa, Artificial Sequence
  source: /note="Description of Artificial Sequence: Synthetic peptide"
EAITTVGAMDY

SEQ ID NO: 16 - protein, 9 aa, Artificial Sequence
  source: /note="Description of Artificial Sequence: Synthetic peptide"
EVLDGAMDY

SEQ ID NO: 17 - protein, 9 aa, Artificial Sequence
  source: /note="Description of Artificial Sequence: Synthetic peptide"
TGYSNLFAY

SEQ ID NO: 18 - protein, 9 aa, Artificial Sequence
  source: /note="Description of Artificial Sequence: Synthetic peptide"
RGYDDYWGY

SEQ ID NO: 19 - protein, 9 aa, Artificial Sequence
  source: /note="Description of Artificial Sequence: Synthetic peptide"
RGHYSAMDY

SEQ ID NO: 20 - protein, 11 aa, Artificial Sequence
  source: /note="Description of Artificial Sequence: Synthetic peptide"
RVGGLEGYFDY

SEQ ID NO: 21 - protein, 11 aa, Artificial Sequence
  source: /note="Description of Artificial Sequence: Synthetic peptide"
RTSENLHNYLA

SEQ ID NO: 22 - protein, 15 aa, Artificial Sequence
  source: /note="Description of Artificial Sequence: Synthetic peptide"
RASESVDNYGISFMN

SEQ ID NO: 23 - protein, 11 aa, Artificial Sequence
  source: /note="Description of Artificial Sequence: Synthetic peptide"
KASQNVGTNVA

SEQ ID NO: 24 - protein, 11 aa, Artificial Sequence
  source: /note="Description of Artificial Sequence: Synthetic peptide"
RASGNIHNYLA

SEQ ID NO: 25 - protein, 15 aa, Artificial Sequence
  source: /note="Description of Artificial Sequence: Synthetic peptide"
RASQSVSTSRFSYMH

SEQ ID NO: 26 - protein, 7 aa, Artificial Sequence
  source: /note="Description of Artificial Sequence: Synthetic peptide"
DAKTLAD

SEQ ID NO: 27 - protein, 7 aa, Artificial Sequence
  source: /note="Description of Artificial Sequence: Synthetic peptide"
AASNQGS

SEQ ID NO: 28 - protein, 7 aa, Artificial Sequence
  source: /note="Description of Artificial Sequence: Synthetic peptide"
SASYRYS

SEQ ID NO: 29 - protein, 7 aa, Artificial Sequence
  source: /note="Description of Artificial Sequence: Synthetic peptide"
NAKTLAD

SEQ ID NO: 30 - protein, 7 aa, Artificial Sequence
  source: /note="Description of Artificial Sequence: Synthetic peptide"
SPSYRYS

SEQ ID NO: 31 - protein, 7 aa, Artificial Sequence
  source: /note="Description of Artificial Sequence: Synthetic peptide"
YASNLES

SEQ ID NO: 32 - protein, 9 aa, Artificial Sequence
  source: /note="Description of Artificial Sequence: Synthetic peptide"
QHFWSSPYT

SEQ ID NO: 33 - protein, 9 aa, Artificial Sequence
  source: /note="Description of Artificial Sequence: Synthetic peptide"
QQSKEVPWT

SEQ ID NO: 34 - protein, 9 aa, Artificial Sequence
  source: /note="Description of Artificial Sequence: Synthetic peptide"
QQYNSYPYT

SEQ ID NO: 35 - protein, 9 aa, Artificial Sequence
  source: /note="Description of Artificial Sequence: Synthetic peptide"
QQYNNYPLT

SEQ ID NO: 36 - protein, 9 aa, Artificial Sequence
  source: /note="Description of Artificial Sequence: Synthetic peptide"
QQYNSYPHT

SEQ ID NO: 37 - protein, 9 aa, Artificial Sequence
  source: /note="Description of Artificial Sequence: Synthetic peptide"
QHSWEIPYT

SEQ ID NO: 38 - protein, 7 aa, Artificial Sequence
  source: /note="Description of Artificial Sequence: Synthetic peptide"
GYTFTDY

SEQ ID NO: 39 - DNA, 360 bp, Artificial Sequence
  source: /note="Description of Artificial Sequence: Synthetic polynucleotide"
gaggtcctgctgcaacagtctggacctgagctggtgaagcctggggcttcagtgaagataccctgcaaggcttctggatacacattcactgactacaacatggactgggtgaagcagagccatggaaagagccttgagtggattggacaaattaatcctaacaatggtggtattttcttcaaccagaagttcaagggcaaggccacattgactgtagacaagtcctccaatacagccttcatggaggtccgcagcctgacatctgaggacactgcagtctattactgtgcaagagaggcaattactacggtaggcgctatggactactggggtcaaggaacctcagtcaccgtctcctca

SEQ ID NO: 40 - protein, 120 aa, Artificial Sequence
  source: /note="Description of Artificial Sequence: Synthetic polypeptide"
EVLLQQSGPELVKPGASVKIPCKASGYTFTDYNMDWVKQSHGKSLEWIGQINPNNGGIFFNQKFKGKATLTVDKSSNTAFMEVRSLTSEDTAVYYCAREAITTVGAMDYWGQGTSVTVSS

SEQ ID NO: 41 - DNA, 354 bp, Artificial Sequence
  source: /note="Description of Artificial Sequence: Synthetic polynucleotide"
caggtccaactgcagcagcctggggctgaactggtgaagcctggggcttcagtgaagctgtcctgcaaggcttctggctacaccttcaccagctactggattcactgggtgaaccagaggcctggacaaggccttgagtggattggagacattaatcctagcaacggccgtagtaagtataatgagaagttcaagaacaaggccacaatgactgcagacaaatcctccaacacagcctacatgcaactcagcagcctgacatctgaggactctgcggtctattactgtgcaagagaggttctggatggtgctatggactactggggtcaaggaacctcagtcaccgtctcctca

SEQ ID NO: 42 - protein, 118 aa, Artificial Sequence
  source: /note="Description of Artificial Sequence: Synthetic polypeptide"
QVQLQQPGAELVKPGASVKLSCKASGYTFTSYWIHWVNQRPGQGLEWIGDINPSNGRSKYNEKFKNKATMTADKSSNTAYMQLSSLTSEDSAVYYCAREVLDGAMDYWGQGTSVTVSS

SEQ ID NO: 43 - DNA, 357 bp, Artificial Sequence
  source: /note="Description of Artificial Sequence: Synthetic polynucleotide"
caggttactctgaaagagtctggccctgggatattgcagccctcccagaccctcagtctgacttgttctttctctgggttttcactgagcacttatggtatgggtgtgacctggattcgtcagccttcaggaaagggtctggagtggctggcacacatttactgggatgatgacaagcgctataacccatccctgaagagccggctcacaatctccaaggatacctccaacaaccaggtattcctcaagatcaccagtgtggacactgcagatactgccacatactactgtgctcaaacggggtatagtaacttgtttgcttactggggccaagggactctggtcactgtctctgca

SEQ ID NO: 44 - protein, 119 aa, Artificial Sequence
  source: /note="Description of Artificial Sequence: Synthetic polypeptide"
QVTLKESGPGILQPSQTLSLTCSFSGFSLSTYGMGVTWIRQPSGKGLEWLAHIYWDDDKRYNPSLKSRLTISKDTSNNQVFLKITSVDTADTATYYCAQTGYSNLFAYWGQGTLVTVSA

SEQ ID NO: 45 - DNA, 357 bp, Artificial Sequence
  source: /note="Description of Artificial Sequence: Synthetic polynucleotide"
caggttactctgaaagagtctggccctgggatattgcagccctcccagaccctcagtctgacttgttctttctctgggttttcactgaacacttatggtatgggtgtgagctggattcgtcagccttcaggaaagggtctggagtggctggcacacatttactgggatgatgacaagcgctataacccatccctgaagagccggctcacaatctccaaggatgcctccaacaaccgggtcttcctcaagatcaccagtgtggacactgcagatactgccacatactactgtgctcaaagaggttatgatgattactggggttactggggccaagggactctggtcactatctctgca

SEQ ID NO: 46 - protein, 119 aa, Artificial Sequence
  source: /note="Description of Artificial Sequence: Synthetic polypeptide"
QVTLKESGPGILQPSQTLSLTCSFSGFSLNTYGMGVSWIRQPSGKGLEWLAHIYWDDDKRYNPSLKSRLTISKDASNNRVFLKITSVDTADTATYYCAQRGYDDYWGYWGQGTLVTISA

SEQ ID NO: 47 - DNA, 360 bp, Artificial Sequence
  source: /note="Description of Artificial Sequence: Synthetic polynucleotide"
gaggtcctgctgcaacagtctggacctgaggtggtgaagcctggggcttcagtgaagataccctgcaaggcttctggatacacattcactgactacaacatggactgggtgaagcagagccatggaaagagccttgagtggattggagagattaatcctaacaatggtggtactttctacaaccagaagttcaagggcaaggccacattgactgtagacaagtcctccagcacagcctacatggagctccgcagcctgacatctgaggacactgcagtctattactgtgcaagagaggcaattactacggtaggcgctatggactactggggtcaaggaacctcagtcaccgtctcctca

SEQ ID NO: 48 - protein, 120 aa, Artificial Sequence
  source: /note="Description of Artificial Sequence: Synthetic polypeptide"
EVLLQQSGPEVVKPGASVKIPCKASGYTFTDYNMDWVKQSHGKSLEWIGEINPNNGGTFYNQKFKGKATLTVDKSSSTAYMELRSLTSEDTAVYYCAREAITTVGAMDYWGQGTSVTVSS

SEQ ID NO: 49 - DNA, 357 bp, Artificial Sequence
  source: /note="Description of Artificial Sequence: Synthetic polynucleotide"
caggttactctgaaagagtctggccctggaatattgcagccctcccagaccctcagtctgacttgttctttctctgggttttcactgagcacttatggtatgggtgtaggctggattcgtcagccttcaggaaagggtctagagtggctggcagacatttggtgggatgacgataagtactataacccatccctgaagagccggctcacaatctccaaggatacctccagcaatgaggtattcctcaagatcgccattgtggacactgcagatactgccacttactactgtgctcgaagaggtcactactctgctatggactactggggtcaaggaacctcagtcaccgtctcctca

SEQ ID NO: 50 - protein, 119 aa, Artificial Sequence
  source: /note="Description of Artificial Sequence: Synthetic polypeptide"
QVTLKESGPGILQPSQTLSLTCSFSGFSLSTYGMGVGWIRQPSGKGLEWLADIWWDDDKYYNPSLKSRLTISKDTSSNEVFLKIAIVDTADTATYYCARRGHYSAMDYWGQGTSVTVSS

SEQ ID NO: 51 - DNA, 363 bp, Artificial Sequence
  source: /note="Description of Artificial Sequence: Synthetic polynucleotide"
caggttactctgaaagagtctggccctgggatattgcagccctcccagaccctcagtctgacttgttctttctctgggttttcactgagcacttctggtatgggtgtgagttggattcgtcagccttcaggaaagggtctggagtggctggcacacaatgactgggatgatgacaagcgctataagtcatccctgaagagccggctcacaatatccaaggatacctccagaaaccaggtattcctcaagatcaccagtgtggacactgcagatactgccacatactactgtgctcgaagagttgggggattagagggctattttgattactggggccaaggcaccactctcacagtctcctca

SEQ ID NO: 52 - protein, 121 aa, Artificial Sequence
  source: /note="Description of Artificial Sequence: Synthetic polypeptide"
QVTLKESGPGILQPSQTLSLTCSFSGFSLSTSGMGVSWIRQPSGKGLEWLAHNDWDDDKRYKSSLKSRLTISKDTSRNQVFLKITSVDTADTATYYCARRVGGLEGYFDYWGQGTTLTVSS

SEQ ID NO: 53 - DNA, 360 bp, Artificial Sequence
  source: /note="Description of Artificial Sequence: Synthetic polynucleotide"
caagtgcaacttgtgcagtcgggtgcggaagtcaaaaagccgggagcgtcggtgaaagtatcgtgtaaagcgtcgggatatacgtttacggactataacatggactgggtacgacaggcaccggggaaatcgttggaatggatcggacagattaatccgaacaatgggggaattttctttaatcagaaattcaaaggacgggcgacgttgacggtcgatacatcgacgaatacggcgtatatggaattgaggtcgcttcgctcggacgatacggcggtctattactgcgccagggaggcgatcacgacggtaggggcgatggattattggggacaggggacgcttgtgacggtatcgtcg

SEQ ID NO: 54 - protein, 120 aa, Artificial Sequence
  source: /note="Description of Artificial Sequence: Synthetic polypeptide"
QVQLVQSGAEVKKPGASVKVSCKASGYTFTDYNMDWVRQAPGKSLEWIGQINPNNGGIFFNQKFKGRATLTVDTSTNTAYMELRSLRSDDTAVYYCAREAITTVGAMDYWGQGTLVTVSS

SEQ ID NO: 55 - DNA, 360 bp, Artificial Sequence
  source: /note="Description of Artificial Sequence: Synthetic polynucleotide"
caagtccagcttgtccagtcgggagcggaagtgaagaaaccggggtcgtcggtcaaagtatcgtgtaaagcgtcgggatatacgtttacggactataacatggattgggtacgacaggctccgggaaaatcattggaatggattggacagattaatccgaataatgggggtatcttctttaatcaaaagtttaaagggagggcgacgttgacggtggacaaatcgacaaatacggcgtatatggaattgtcgtcgcttcggtcggaggacacggcggtgtattactgcgcgagggaggcgatcacgacggtcggggcgatggattattggggacagggaacgcttgtgacggtatcgtcg

SEQ ID NO: 56 - protein, 120 aa, Artificial Sequence
  source: /note="Description of Artificial Sequence: Synthetic polypeptide"
QVQLVQSGAEVKKPGSSVKVSCKASGYTFTDYNMDWVRQAPGKSLEWIGQINPNNGGIFFNQKFKGRATLTVDKSTNTAYMELSSLRSEDTAVYYCAREAITTVGAMDYWGQGTLVTVSS

SEQ ID NO: 57 - DNA, 360 bp, Artificial Sequence
  source: /note="Description of Artificial Sequence: Synthetic polynucleotide"
caggtccagcttgtgcaatcgggagcggaagtgaagaaaccgggagcgtcggtaaaagtctcgtgcaaagcgtcggggtatacgtttacggactataacatggactgggtgcgccaagcgcctggacagggtcttgaatggatggggcagattaatccgaataatggagggatcttctttaatcagaaattcaaaggaagggtaacgctgacgacagacacgtcaacatcgacggcctatatggaattgcggtcgttgcgatcagatgatacggcggtctactattgtgcgagggaggcgattacgacggtgggagcgatggattattggggacaggggacgttggtaacggtatcgtcg

SEQ ID NO: 58 - protein, 120 aa, Artificial Sequence
  source: /note="Description of Artificial Sequence: Synthetic polypeptide"
QVQLVQSGAEVKKPGASVKVSCKASGYTFTDYNMDWVRQAPGQGLEWMGQINPNNGGIFFNQKFKGRVTLTTDTSTSTAYMELRSLRSDDTAVYYCAREAITTVGAMDYWGQGTLVTVSS

SEQ ID NO: 59 - DNA, 360 bp, Artificial Sequence
  source: /note="Description of Artificial Sequence: Synthetic polynucleotide"
caggtccagcttgtgcaatcgggagcggaagtgaagaaaccgggagcgtcggtaaaagtctcgtgcaaagcgtcggggtatacgtttacggactataacatggactgggtgcgccaagcgcctggacagagccttgaatggatggggcagattaatccgaataatggagggatcttctttaatcagaaattccagggaagggtaacgctgacgacagacacgtcaacatcgacggcctatatggaattgcggtcgttgcgatcagatgatacggcggtctactattgtgcgagggaggcgattacgacggtgggagcgatggattattggggacaggggacgttggtaacggtatcgtcg

SEQ ID NO: 60 - protein, 120 aa, Artificial Sequence
  source: /note="Description of Artificial Sequence: Synthetic polypeptide"
QVQLVQSGAEVKKPGASVKVSCKASGYTFTDYNMDWVRQAPGQSLEWMGQINPNNGGIFFNQKFQGRVTLTTDTSTSTAYMELRSLRSDDTAVYYCAREAITTVGAMDYWGQGTLVTVSS

SEQ ID NO: 61 - DNA, 360 bp, Artificial Sequence
  source: /note="Description of Artificial Sequence: Synthetic polynucleotide"
caggtccagcttgtgcaatcgggagcggaagtgaagaaaccgggagcgtcggtaaaagtctcgtgcaaagcgtcggggtatacgtttacggactataacatggactgggtgcgccaagcgcctggacagggtcttgaatggatggggcagattaatccgaataatggagggatcttctttaatcagaaattccagggaagggtaacgctgacgacagacacgtcaacatcgacggcctatatggaattgcggtcgttgcgatcagatgatacggcggtctactattgtgcgagggaggcgattacgacggtgggagcgatggattattggggacaggggacgttggtaacggtatcgtcg

SEQ ID NO: 62 - protein, 120 aa, Artificial Sequence
  source: /note="Description of Artificial Sequence: Synthetic polypeptide"
QVQLVQSGAEVKKPGASVKVSCKASGYTFTDYNMDWVRQAPGQGLEWMGQINPNNGGIFFNQKFQGRVTLTTDTSTSTAYMELRSLRSDDTAVYYCAREAITTVGAMDYWGQGTLVTVSS

SEQ ID NO: 63 - DNA, 360 bp, Artificial Sequence
  source: /note="Description of Artificial Sequence: Synthetic polynucleotide"
caagtacagcttgtacagtcgggagcggaagtcaagaaaccgggatcgtcggtcaaagtgtcgtgtaaagcgtcgggatatacgtttagcgactataacatggattgggtgcgacaagcgcctgggcagggacttgaatggatgggtcagatcaatccgaataatgggggaatctttttcaatcagaagtttaaagggagggtaacgctgacggcggataaaagcacgtcaacggcgtatatggagttgtcgtcgttgcggtcggaggacacggcggtctattactgcgcgagggaagcgattacgacggtgggagcgatggattattgggggcagggaacgcttgtaacggtgtcatcg

SEQ ID NO: 64 - protein, 120 aa, Artificial Sequence
  source: /note="Description of Artificial Sequence: Synthetic polypeptide"
QVQLVQSGAEVKKPGSSVKVSCKASGYTFSDYNMDWVRQAPGQGLEWMGQINPNNGGIFFNQKFKGRVTLTADKSTSTAYMELSSLRSEDTAVYYCAREAITTVGAMDYWGQGTLVTVSS

SEQ ID NO: 65 - DNA, 360 bp, Artificial Sequence
  source: /note="Description of Artificial Sequence: Synthetic polynucleotide"
caagtacagcttgtacagtcgggagcggaagtcaagaaaccgggatcgtcggtcaaagtgtcgtgtaaagcgtcgggatatacgtttagcgactataacatggattgggtgcgacaagcgcctgggcagggacttgaatggatgggtcagatcaatccgaataatgggggaatctttttcaatcagaagtttcaggggagggtaacgctgacggcggataaaagcacgtcaacggcgtatatggagttgtcgtcgttgcggtcggaggacacggcggtctattactgcgcgagggaagcgattacgacggtgggagcgatggattattgggggcagggaacgcttgtaacggtgtcatcg

SEQ ID NO: 66 - protein, 120 aa, Artificial Sequence
  source: /note="Description of Artificial Sequence: Synthetic polypeptide"
QVQLVQSGAEVKKPGSSVKVSCKASGYTFSDYNMDWVRQAPGQGLEWMGQINPNNGGIFFNQKFQGRVTLTADKSTSTAYMELSSLRSEDTAVYYCAREAITTVGAMDYWGQGTLVTVSS

SEQ ID NO: 67 - DNA, 357 bp, Artificial Sequence
  source: /note="Description of Artificial Sequence: Synthetic polynucleotide"
caggtgactttgaaagaatccggtcccgcattggtaaagccaacccagacacttacgctcacatgtacattttccggattcagcttgaacacttacgggatgggagtgtcgtggattcggcaacctccggggaaggctctggagtggctggcgcacatctactgggatgatgacaaaaggtataacccctcacttaaaacgagactgacgatctcgaaggacacaagcaagaatcaggtcgtcctcacgattacgaatgtagacccggtggatactgccgtctattactgcgcgcaacgcgggtatgatgactactggggatattggggtcagggcaccctcgtgaccatctcgtca

SEQ ID NO: 68 - protein, 119 aa, Artificial Sequence
  source: /note="Description of Artificial Sequence: Synthetic polypeptide"
QVTLKESGPALVKPTQTLTLTCTFSGFSLNTYGMGVSWIRQPPGKALEWLAHIYWDDDKRYNPSLKTRLTISKDTSKNQVVLTITNVDPVDTAVYYCAQRGYDDYWGYWGQGTLVTISS

SEQ ID NO: 69 - DNA, 357 bp, Artificial Sequence
  source: /note="Description of Artificial Sequence: Synthetic polynucleotide"
caagtaacgctcaaggagtccggacccaccttggtgaagccgacgcagaccttgactcttacgtgcactttctcggggttttcactgaatacgtacgggatgggtgtctcatggatcaggcaacctccggggaaaggattggaatggctggcgcacatctactgggatgacgataagagatataacccaagcctcaagtcgcggctcaccattacaaaagatacatcgaaaaatcaggtcgtacttactatcacgaacatggaccccgtggacacagcaacatattactgtgcccagcgcggctatgacgattattggggttactggggacagggaacactggtcacggtgtccagc

SEQ ID NO: 70 - protein, 119 aa, Artificial Sequence
  source: /note="Description of Artificial Sequence: Synthetic polypeptide"
QVTLKESGPTLVKPTQTLTLTCTFSGFSLNTYGMGVSWIRQPPGKGLEWLAHIYWDDDKRYNPSLKSRLTITKDTSKNQVVLTITNMDPVDTATYYCAQRGYDDYWGYWGQGTLVTVSS

SEQ ID NO: 71 - DNA, 357 bp, Artificial Sequence
  source: /note="Description of Artificial Sequence: Synthetic polynucleotide"
cagatcactttgaaagaaagcggaccgaccttggtcaagcccacacaaaccctcacgctcacgtgtacattttcggggttctcgctttcaacttacgggatgggagtagggtggattcgccagccgcctggtaaagcgttggagtggcttgcagacatctggtgggacgacgataagtactataatccctcgctcaagtccagactgaccatcacgaaagatacgagcaagaaccaggtcgtgctgacaatgactaacatggacccagtggatacggctacatattactgcgccaggcggggtcactactcagcgatggattattggggccagggaacactggtaacggtgtcgtcc

SEQ ID NO: 72 - protein, 119 aa, Artificial Sequence
  source: /note="Description of Artificial Sequence: Synthetic polypeptide"
QITLKESGPTLVKPTQTLTLTCTFSGFSLSTYGMGVGWIRQPPGKALEWLADIWWDDDKYYNPSLKSRLTITKDTSKNQVVLTMTNMDPVDTATYYCARRGHYSAMDYWGQGTLVTVSS

SEQ ID NO: 73 - DNA, 357 bp, Artificial Sequence
  source: /note="Description of Artificial Sequence: Synthetic polynucleotide"
caagtgactctcaaggagtccggacccgccctggtcaaaccaacgcagacactgacgctcacatgcaccttcagcggattttcgttgtcaacgtacggcatgggtgtggggtggattcgccagcctccggggaaagcccttgaatggttggcggacatctggtgggatgatgacaagtactataatccctcacttaagtcacggttgacgatctcgaaagacaccagcaagaaccaggtagtgctgacaatgactaacatggacccggtcgatacagcggtctactattgtgctagaaggggacactactccgcaatggattattggggtcaggggacgctcgtaaccgtgtcgtcg

SEQ ID NO: 74 - protein, 119 aa, Artificial Sequence
  source: /note="Description of Artificial Sequence: Synthetic polypeptide"
QVTLKESGPALVKPTQTLTLTCTFSGFSLSTYGMGVGWIRQPPGKALEWLADIWWDDDKYYNPSLKSRLTISKDTSKNQVVLTMTNMDPVDTAVYYCARRGHYSAMDYWGQGTLVTVSS

SEQ ID NO: 75 - DNA, 321 bp, Artificial Sequence
  source: /note="Description of Artificial Sequence: Synthetic polynucleotide"
gacatccagatgactcagtctccagcctccctatctgcatctgtgggagaaactgtcaccatcacatgtcgaacaagtgagaatcttcacaattatttagcatggtatcagcagaaacagggaaaatctcctcagctcctggtctatgatgcaaaaaccttagcagatggtgtgccatcaaggttcagtggcagtggatcaggaacacaatattctctcaagatcaacagcctgcagcctgaagattttgggagttattactgtcaacatttttggagtagtccttacacgttcggaggggggaccaagctggaaataaaa

SEQ ID NO: 76 - protein, 107 aa, Artificial Sequence
  source: /note="Description of Artificial Sequence: Synthetic polypeptide"
DIQMTQSPASLSASVGETVTITCRTSENLHNYLAWYQQKQGKSPQLLVYDAKTLADGVPSRFSGSGSGTQYSLKINSLQPEDFGSYYCQHFWSSPYTFGGGTKLEIK

SEQ ID NO: 77 - DNA, 333 bp, Artificial Sequence
  source: /note="Description of Artificial Sequence: Synthetic polynucleotide"
gacattgtgttgacccaatctccagcttctttggctgtgtctctagggcagagggccaccatctcctgcagagccagcgaaagtgttgataattatggcattagttttatgaactggttccaacagaaaccaggacagccacccaaactcctcatctatgctgcatccaaccaaggctccggggtccctgccaggtttagtggcagtgggtctgggacagacttcagcctcaacatccatcctatggaggaggatgatactgcaatgtatttctgtcagcaaagtaaggaggttccgtggacgttcggtggaggctccaagctggaaatcaaa

SEQ ID NO: 78 - protein, 111 aa, Artificial Sequence
  source: /note="Description of Artificial Sequence: Synthetic polypeptide"
DIVLTQSPASLAVSLGQRATISCRASESVDNYGISFMNWFQQKPGQPPKLLIYAASNQGSGVPARFSGSGSGTDFSLNIHPMEEDDTAMYFCQQSKEVPWTFGGGSKLEIK

SEQ ID NO: 79 - DNA, 321 bp, Artificial Sequence
  source: /note="Description of Artificial Sequence: Synthetic polynucleotide"
gacattgtgatgacccagtctcaaaaattcatgtccacatcagtaggagacagggtcagcgtcacctgcaaggccagtcagaatgtgggtactaatgtagcctggtatcaacagaaattaggacaatctcctaaaacactgatttactcggcatcctaccggtacagtggagtccctgatcgcttcacaggcagtggatctgggacagatttcactctcaccatcagcaatgtgcagtctgaagacttggcagagtatttctgtcagcaatataacagctatccgtacacgttcggaggggggaccaagctggaaataaaa

SEQ ID NO: 80 - protein, 107 aa, Artificial Sequence
  source: /note="Description of Artificial Sequence: Synthetic polypeptide"
DIVMTQSQKFMSTSVGDRVSVTCKASQNVGTNVAWYQQKLGQSPKTLIYSASYRYSGVPDRFTGSGSGTDFTLTISNVQSEDLAEYFCQQYNSYPYTFGGGTKLEIK

SEQ ID NO: 81 - DNA, 321 bp, Artificial Sequence
  source: /note="Description of Artificial Sequence: Synthetic polynucleotide"
gacattgtgatgacccagtctcaaaaattcatgtccacatcagtaggagacagggtcagcgtcacctgcaaggccagtcagaatgtgggtactaatgtagcctggtttcaacagaaaccaggtcaatctcctaaagcactgatttactcggcatcttaccggtacagtggagtccctgatcgcttcacaggcagtggatctgggacagatttcattctcaccatcagcaatgtgcagtctgaagacctggcagagtatttctgtcagcaatataacaactatcctctcacgttcggtgctgggaccaagctggagctgaaa

SEQ ID NO: 82 - protein, 107 aa, Artificial Sequence
  source: /note="Description of Artificial Sequence: Synthetic polypeptide"
DIVMTQSQKFMSTSVGDRVSVTCKASQNVGTNVAWFQQKPGQSPKALIYSASYRYSGVPDRFTGSGSGTDFILTISNVQSEDLAEYFCQQYNNYPLTFGAGTKLELK

SEQ ID NO: 83 - DNA, 321 bp, Artificial Sequence
  source: /note="Description of Artificial Sequence: Synthetic polynucleotide"
gacatccagatgactcagtctccagcctccctatctgcatctgtgggagaaactgtcaccatcacatgtcgagcaagtgggaatattcacaattatttagcatggtatcagcagaaacagggaaaatctcctcagctcctggtctataatgcaaaaaccttagcagatggtgtgccatcaaggttcagtggcagtggatcaggaacacaatattctctcaagatcaacagcctgcagcctgaagattttgggagttattactgtcaacatttttggagttctccttacacgttcggaggggggaccaagctggaaataaaa

SEQ ID NO: 84 - protein, 107 aa, Artificial Sequence
  source: /note="Description of Artificial Sequence: Synthetic polypeptide"
DIQMTQSPASLSASVGETVTITCRASGNIHNYLAWYQQKQGKSPQLLVYNAKTLADGVPSRFSGSGSGTQYSLKINSLQPEDFGSYYCQHFWSSPYTFGGGTKLEIK

SEQ ID NO: 85 - DNA, 321 bp, Artificial Sequence
  source: /note="Description of Artificial Sequence: Synthetic polynucleotide"
gacattgtaatgacccagtctcaaaaattcatgtccacatcagtaggagacagggtcagcgtcacctgcaaggccagtcagaatgtgggtactaatgtagcctggtatcaacagaaaccagggcaatctcctaaagcactgatttactcgccatcctaccggtacagtggagtccctgatcgcttcacaggcagtggatctgggacagatttcactctcaccatcagcaatgtgcagtctgaagacttggcagaatatttctgtcagcaatataacagctatcctcacacgttcggaggggggaccaagctggaaatgaaa

SEQ ID NO: 86 - protein, 107 aa, Artificial Sequence
  source: /note="Description of Artificial Sequence: Synthetic polypeptide"
DIVMTQSQKFMSTSVGDRVSVTCKASQNVGTNVAWYQQKPGQSPKALIYSPSYRYSGVPDRFTGSGSGTDFTLTISNVQSEDLAEYFCQQYNSYPHTFGGGTKLEMK

SEQ ID NO: 87 - DNA, 333 bp, Artificial Sequence
  source: /note="Description of Artificial Sequence: Synthetic polynucleotide"
gacattgtgctgacacagtctcctgcttccttagctgtatctctggggcagagggccaccatctcatgcagggccagccaaagtgtcagtacatctaggtttagttatatgcactggttccaacagaaaccaggacaggcacccaaactcctcatcaagtatgcatccaacctagaatctggggtccctgccaggttcagtggcagtgggtctgggacagacttcaccctcaacatccatcctgtggagggggaggatactgcaacatattactgtcagcacagttgggagattccgtacacgttcggaggggggaccaagctggaaataaaa

SEQ ID NO: 88 - protein, 111 aa, Artificial Sequence
  source: /note="Description of Artificial Sequence: Synthetic polypeptide"
DIVLTQSPASLAVSLGQRATISCRASQSVSTSRFSYMHWFQQKPGQAPKLLIKYASNLESGVPARFSGSGSGTDFTLNIHPVEGEDTATYYCQHSWEIPYTFGGGTKLEIK

SEQ ID NO: 89 - DNA, 321 bp, Artificial Sequence
  source: /note="Description of Artificial Sequence: Synthetic polynucleotide"
gacatccaaatgacccagtcgccgtcgtcgctttcagcgtcggtaggggatcgggtcacaattacgtgccgaacgtcagagaatttgcataactacctcgcgtggtatcagcagaagcccgggaagtcaccgaaactccttgtctacgatgcgaaaacgctggcggatggagtgccgtcgagattctcgggaagcggatccggtacggactatacgcttacgatctcatcgctccagcccgaggactttgcgacgtactattgtcagcatttttggtcgtcgccctacacatttgggcaggggaccaagttggaaatcaag

SEQ ID NO: 90 - protein, 107 aa, Artificial Sequence
  source: /note="Description of Artificial Sequence: Synthetic polypeptide"
DIQMTQSPSSLSASVGDRVTITCRTSENLHNYLAWYQQKPGKSPKLLVYDAKTLADGVPSRFSGSGSGTDYTLTISSLQPEDFATYYCQHFWSSPYTFGQGTKLEIK

SEQ ID NO: 91 - DNA, 321 bp, Artificial Sequence
  source: /note="Description of Artificial Sequence: Synthetic polynucleotide"
gacatccaaatgacccagtcgccgtcgtcgctttcagcgtcggtaggggatcgggtcacaattacgtgccgaacgtcagagaatttgcataactacctcgcgtggtatcagcagaagcccgggaaggccccgaaactccttatctacgatgcgaaaacgctggcggatggagtgccgtcgagattctcgggaagcggatccggtacggactatacgcttacgatctcatcgctccagcccgaggactttgcgacgtactattgtcagcatttttggtcgtcgccctacacatttgggcaggggaccaagttggaaatcaag

SEQ ID NO: 92 - protein, 107 aa, Artificial Sequence
  source: /note="Description of Artificial Sequence: Synthetic polypeptide"
DIQMTQSPSSLSASVGDRVTITCRTSENLHNYLAWYQQKPGKAPKLLIYDAKTLADGVPSRFSGSGSGTDYTLTISSLQPEDFATYYCQHFWSSPYTFGQGTKLEIK

SEQ ID NO: 93 - DNA, 321 bp, Artificial Sequence
  source: /note="Description of Artificial Sequence: Synthetic polynucleotide"
gacatccaaatgacccagtcgccgtcgtcgctttcagcgtcggtaggggatcgggtcacaattacgtgccgaacgtcagagaatttgcataactacctcgcgtggtatcagcagaagcccgggaagtcaccgaaactccttatctacgatgcgaaaacgctggcggatggagtgccgtcgagattctcgggaagcggatccggtacggactatacgcttacgatctcatcgctccagcccgaggactttgcgacgtactattgtcagcatttttggtcgtcgccctacacatttgggcaggggaccaagttggaaatcaag

SEQ ID NO: 94 - protein, 107 aa, Artificial Sequence
  source: /note="Description of Artificial Sequence: Synthetic polypeptide"
DIQMTQSPSSLSASVGDRVTITCRTSENLHNYLAWYQQKPGKSPKLLIYDAKTLADGVPSRFSGSGSGTDYTLTISSLQPEDFATYYCQHFWSSPYTFGQGTKLEIK

SEQ ID NO: 95 - DNA, 321 bp, Artificial Sequence
  source: /note="Description of Artificial Sequence: Synthetic polynucleotide"
gacatccaaatgacccaatcgccctcctccctctccgcatcagtaggggaccgcgtcacaattacttgcaaagcgtcgcagaacgtcggaacgaatgtggcgtggtttcagcagaagcccggaaaagctccgaagagcttgatctactcggcctcatataggtattcgggtgtgccgagccggtttagcgggtcggggtcaggtactgatttcacgctcacaatttcatcgttgcagccagaagatttcgccacatattactgtcagcagtacaacaattaccctctgacgttcggccagggaaccaaacttgagatcaag

SEQ ID NO: 96 - protein, 107 aa, Artificial Sequence
  source: /note="Description of Artificial Sequence: Synthetic polypeptide"
DIQMTQSPSSLSASVGDRVTITCKASQNVGTNVAWFQQKPGKAPKSLIYSASYRYSGVPSRFSGSGSGTDFTLTISSLQPEDFATYYCQQYNNYPLTFGQGTKLEIK

SEQ ID NO: 97 - DNA, 321 bp, Artificial Sequence
  source: /note="Description of Artificial Sequence: Synthetic polynucleotide"
gatatccagatgacacagtcaccctcgtcgctctcagcttccgtaggcgacagggtcactattacgtgtaaagcatcacagaacgtcggaacgaatgtggcgtggtttcagcagaagcccgggaagagccccaaagcgcttatctactccccgtcgtatcggtattccggtgtgccaagcagattttcggggtcaggttcgggaactgactttaccctgaccatctcgtccctccaaccggaagatttcgccacgtacttctgccagcagtacaacagctatcctcacacattcggacaagggacaaagttggagattaaa

SEQ ID NO: 98 - protein, 107 aa, Artificial Sequence
  source: /note="Description of Artificial Sequence: Synthetic polypeptide"
DIQMTQSPSSLSASVGDRVTITCKASQNVGTNVAWFQQKPGKSPKALIYSPSYRYSGVPSRFSGSGSGTDFTLTISSLQPEDFATYFCQQYNSYPHTFGQGTKLEIK

SEQ ID NO: 99 - DNA, 1332 bp, Artificial Sequence
  source: /note="Description of Artificial Sequence: Synthetic polynucleotide"
gaggtcctgctgcaacagtctggacctgagctggtgaagcctggggcttcagtgaagataccctgcaaggcttctggatacacattcactgactacaacatggactgggtgaagcagagccatggaaagagccttgagtggattggacaaattaatcctaacaatggtggtattttcttcaaccagaagttcaagggcaaggccacattgactgtagacaagtcctccaatacagccttcatggaggtccgcagcctgacatctgaggacactgcagtctattactgtgcaagagaggcaattactacggtaggcgctatggactactggggtcaaggaacctcagtcaccgtctcctcagccaaaacgacacccccatctgtctatccactggcccctggatctgctgcccaaactaactccatggtgaccctgggatgcctggtcaagggctatttccctgagccagtgacagtgacctggaactctggatccctgtccagcggtgtgcacaccttcccagctgtcctgcagtctgacctctacactctgagcagctcagtgactgtcccctccagcacctggcccagcgagaccgtcacctgcaacgttgcccacccggccagcagcaccaaggtggacaagaaaattgtgcccagggattgtggttgtaagccttgcatatgtacagtcccagaagtatcatctgtcttcatcttccccccaaagcccaaggatgtgctcaccattactctgactcctaaggtcacgtgtgttgtggtagacatcagcaaggatgatcccgaggtccagttcagctggtttgtagatgatgtggaggtgcacacagctcagacgcaaccccgggaggagcagttcaacagcactttccgctcagtcagtgaacttcccatcatgcaccaggactggctcaatggcaaggagttcaaatgcagggtcaacagtgcagctttccctgcccccatcgagaaaaccatctccaaaaccaaaggcagaccgaaggctccacaggtgtacaccattccacctcccaaggagcagatggccaaggataaagtcagtctgacctgcatgataacagacttcttccctgaagacattactgtggagtggcagtggaatgggcagccagcggagaactacaagaacactcagcccatcatggacacagatggctcttacttcgtctacagcaagctcaatgtgcagaagagcaactgggaggcaggaaatactttcacctgctctgtgttacatgagggcctgcacaaccaccatactgagaagagcctctcccactctcctggtaaa

SEQ ID NO: 100 - protein, 444 aa, Artificial Sequence
  source: /note="Description of Artificial Sequence: Synthetic polypeptide"
EVLLQQSGPELVKPGASVKIPCKASGYTFTDYNMDWVKQSHGKSLEWIGQINPNNGGIFFNQKFKGKATLTVDKSSNTAFMEVRSLTSEDTAVYYCAREAITTVGAMDYWGQGTSVTVSSAKTTPPSVYPLAPGSAAQTNSMVTLGCLVKGYFPEPVTVTWNSGSLSSGVHTFPAVLQSDLYTLSSSVTVPSSTWPSETVTCNVAHPASSTKVDKKIVPRDCGCKPCICTVPEVSSVFIFPPKPKDVLTITLTPKVTCVVVDISKDDPEVQFSWFVDDVEVHTAQTQPREEQFNSTFRSVSELPIMHQDWLNGKEFKCRVNSAAFPAPIEKTISKTKGRPKAPQVYTIPPPKEQMAKDKVSLTCMITDFFPEDITVEWQWNGQPAENYKNTQPIMDTDGSYFVYSKLNVQKSNWEAGNTFTCSVLHEGLHNHHTEKSLSHSPGK

SEQ ID NO: 101 - DNA, 642 bp, Artificial Sequence
  source: /note="Description of Artificial Sequence: Synthetic polynucleotide"
gacatccagatgactcagtctccagcctccctatctgcatctgtgggagaaactgtcaccatcacatgtcgaacaagtgagaatcttcacaattatttagcatggtatcagcagaaacagggaaaatctcctcagctcctggtctatgatgcaaaaaccttagcagatggtgtgccatcaaggttcagtggcagtggatcaggaacacaatattctctcaagatcaacagcctgcagcctgaagattttgggagttattactgtcaacatttttggagtagtccttacacgttcggaggggggaccaagctggaaataaaacgggctgatgctgcaccaactgtatccatcttcccaccatccagtgagcagttaacatctggaggtgcctcagtcgtgtgcttcttgaacaacttctaccccaaagacatcaatgtcaagtggaagattgatggcagtgaacgacaaaatggcgtcctgaacagttggactgatcaggacagcaaagacagcacctacagcatgagcagcaccctcacgttgaccaaggacgagtatgaacgacataacagctatacctgtgaggccactcacaagacatcaacttcacccattgtcaagagcttcaacaggaatgagtgt

SEQ ID NO: 102 - protein, 214 aa, Artificial Sequence
  source: /note="Description of Artificial Sequence: Synthetic polypeptide"
DIQMTQSPASLSASVGETVTITCRTSENLHNYLAWYQQKQGKSPQLLVYDAKTLADGVPSRFSGSGSGTQYSLKINSLQPEDFGSYYCQHFWSSPYTFGGGTKLEIKRADAAPTVSIFPPSSEQLTSGGASVVCFLNNFYPKDINVKWKIDGSERQNGVLNSWTDQDSKDSTYSMSSTLTLTKDEYERHNSYTCEATHKTSTSPIVKSFNRNEC

SEQ ID NO: 103 - DNA, 1326 bp, Artificial Sequence
  source: /note="Description of Artificial Sequence: Synthetic polynucleotide"
caggtccaactgcagcagcctggggctgaactggtgaagcctggggcttcagtgaagctgtcctgcaaggcttctggctacaccttcaccagctactggattcactgggtgaaccagaggcctggacaaggccttgagtggattggagacattaatcctagcaacggccgtagtaagtataatgagaagttcaagaacaaggccacaatgactgcagacaaatcctccaacacagcctacatgcaactcagcagcctgacatctgaggactctgcggtctattactgtgcaagagaggttctggatggtgctatggactactggggtcaaggaacctcagtcaccgtctcctcagccaaaacgacacccccatctgtctatccactggcccctggatctgctgcccaaactaactccatggtgaccctgggatgcctggtcaagggctatttccctgagccagtgacagtgacctggaactctggatccctgtccagcggtgtgcacaccttcccagctgtcctgcagtctgacctctacactctgagcagctcagtgactgtcccctccagcacctggcccagcgagaccgtcacctgcaacgttgcccacccggccagcagcaccaaggtggacaagaaaattgtgcccagggattgtggttgtaagccttgcatatgtacagtcccagaagtatcatctgtcttcatcttccccccaaagcccaaggatgtgctcaccattactctgactcctaaggtcacgtgtgttgtggtagacatcagcaaggatgatcccgaggtccagttcagctggtttgtagatgatgtggaggtgcacacagctcagacgcaaccccgggaggagcagttcaacagcactttccgctcagtcagtgaacttcccatcatgcaccaggactggctcaatggcaaggagttcaaatgcagggtcaacagtgcagctttccctgcccccatcgagaaaaccatctccaaaaccaaaggcagaccgaaggctccacaggtgtacaccattccacctcccaaggagcagatggccaaggataaagtcagtctgacctgcatgataacagacttcttccctgaagacattactgtggagtggcagtggaatgggcagccagcggagaactacaagaacactcagcccatcatggacacagatggctcttacttcgtctacagcaagctcaatgtgcagaagagcaactgggaggcaggaaatactttcacctgctctgtgttacatgagggcctgcacaaccaccatactgagaagagcctctcccactctcctggtaaa

SEQ ID NO: 104 - protein, 442 aa, Artificial Sequence
  source: /note="Description of Artificial Sequence: Synthetic polypeptide"
QVQLQQPGAELVKPGASVKLSCKASGYTFTSYWIHWVNQRPGQGLEWIGDINPSNGRSKYNEKFKNKATMTADKSSNTAYMQLSSLTSEDSAVYYCAREVLDGAMDYWGQGTSVTVSSAKTTPPSVYPLAPGSAAQTNSMVTLGCLVKGYFPEPVTVTWNSGSLSSGVHTFPAVLQSDLYTLSSSVTVPSSTWPSETVTCNVAHPASSTKVDKKIVPRDCGCKPCICTVPEVSSVFIFPPKPKDVLTITLTPKVTCVVVDISKDDPEVQFSWFVDDVEVHTAQTQPREEQFNSTFRSVSELPIMHQDWLNGKEFKCRVNSAAFPAPIEKTISKTKGRPKAPQVYTIPPPKEQMAKDKVSLTCMITDFFPEDITVEWQWNGQPAENYKNTQPIMDTDGSYFVYSKLNVQKSNWEAGNTFTCSVLHEGLHNHHTEKSLSHSPGK

SEQ ID NO: 105 - DNA, 654 bp, Artificial Sequence
  source: /note="Description of Artificial Sequence: Synthetic polynucleotide"
gacattgtgttgacccaatctccagcttctttggctgtgtctctagggcagagggccaccatctcctgcagagccagcgaaagtgttgataattatggcattagttttatgaactggttccaacagaaaccaggacagccacccaaactcctcatctatgctgcatccaaccaaggctccggggtccctgccaggtttagtggcagtgggtctgggacagacttcagcctcaacatccatcctatggaggaggatgatactgcaatgtatttctgtcagcaaagtaaggaggttccgtggacgttcggtggaggctccaagctggaaatcaaacgggctgatgctgcaccaactgtatccatcttcccaccatccagtgagcagttaacatctggaggtgcctcagtcgtgtgcttcttgaacaacttctaccccaaagacatcaatgtcaagtggaagattgatggcagtgaacgacaaaatggcgtcctgaacagttggactgatcaggacagcaaagacagcacctacagcatgagcagcaccctcacgttgaccaaggacgagtatgaacgacataacagctatacctgtgaggccactcacaagacatcaacttcacccattgtcaagagcttcaacaggaatgagtgt

SEQ ID NO: 106 - protein, 218 aa, Artificial Sequence
  source: /note="Description of Artificial Sequence: Synthetic polypeptide"
DIVLTQSPASLAVSLGQRATISCRASESVDNYGISFMNWFQQKPGQPPKLLIYAASNQGSGVPARFSGSGSGTDFSLNIHPMEEDDTAMYFCQQSKEVPWTFGGGSKLEIKRADAAPTVSIFPPSSEQLTSGGASVVCFLNNFYPKDINVKWKIDGSERQNGVLNSWTDQDSKDSTYSMSSTLTLTKDEYERHNSYTCEATHKTSTSPIVKSFNRNEC

SEQ ID NO: 107 - DNA, 1329 bp, Artificial Sequence
  source: /note="Description of Artificial Sequence: Synthetic polynucleotide"
caggttactctgaaagagtctggccctgggatattgcagccctcccagaccctcagtctgacttgttctttctctgggttttcactgagcacttatggtatgggtgtgacctggattcgtcagccttcaggaaagggtctggagtggctggcacacatttactgggatgatgacaagcgctataacccatccctgaagagccggctcacaatctccaaggatacctccaacaaccaggtattcctcaagatcaccagtgtggacactgcagatactgccacatactactgtgctcaaacggggtatagtaacttgtttgcttactggggccaagggactctggtcactgtctctgcagccaaaacgacacccccatctgtctatccactggcccctggatctgctgcccaaactaactccatggtgaccctgggatgcctggtcaagggctatttccctgagccagtgacagtgacctggaactctggatccctgtccagcggtgtgcacaccttcccagctgtcctgcagtctgacctctacactctgagcagctcagtgactgtcccctccagcacctggcccagcgagaccgtcacctgcaacgttgcccacccggccagcagcaccaaggtggacaagaaaattgtgcccagggattgtggttgtaagccttgcatatgtacagtcccagaagtatcatctgtcttcatcttccccccaaagcccaaggatgtgctcaccattactctgactcctaaggtcacgtgtgttgtggtagacatcagcaaggatgatcccgaggtccagttcagctggtttgtagatgatgtggaggtgcacacagctcagacgcaaccccgggaggagcagttcaacagcactttccgctcagtcagtgaacttcccatcatgcaccaggactggctcaatggcaaggagttcaaatgcagggtcaacagtgcagctttccctgcccccatcgagaaaaccatctccaaaaccaaaggcagaccgaaggctccacaggtgtacaccattccacctcccaaggagcagatggccaaggataaagtcagtctgacctgcatgataacagacttcttccctgaagacattactgtggagtggcagtggaatgggcagccagcggagaactacaagaacactcagcccatcatggacacagatggctcttacttcgtctacagcaagctcaatgtgcagaagagcaactgggaggcaggaaatactttcacctgctctgtgttacatgagggcctgcacaaccaccatactgagaagagcctctcccactctcctggtaaa

SEQ ID NO: 108 - protein, 443 aa, Artificial Sequence
  source: /note="Description of Artificial Sequence: Synthetic polypeptide"
QVTLKESGPGILQPSQTLSLTCSFSGFSLSTYGMGVTWIRQPSGKGLEWLAHIYWDDDKRYNPSLKSRLTISKDTSNNQVFLKITSVDTADTATYYCAQTGYSNLFAYWGQGTLVTVSAAKTTPPSVYPLAPGSAAQTNSMVTLGCLVKGYFPEPVTVTWNSGSLSSGVHTFPAVLQSDLYTLSSSVTVPSSTWPSETVTCNVAHPASSTKVDKKIVPRDCGCKPCICTVPEVSSVFIFPPKPKDVLTITLTPKVTCVVVDISKDDPEVQFSWFVDDVEVHTAQTQPREEQFNSTFRSVSELPIMHQDWLNGKEFKCRVNSAAFPAPIEKTISKTKGRPKAPQVYTIPPPKEQMAKDKVSLTCMITDFFPEDITVEWQWNGQPAENYKNTQPIMDTDGSYFVYSKLNVQKSNWEAGNTFTCSVLHEGLHNHHTEKSLSHSPGK

SEQ ID NO: 109 - DNA, 642 bp, Artificial Sequence
  source: /note="Description of Artificial Sequence: Synthetic polynucleotide"
gacattgtgatgacccagtctcaaaaattcatgtccacatcagtaggagacagggtcagcgtcacctgcaaggccagtcagaatgtgggtactaatgtagcctggtatcaacagaaattaggacaatctcctaaaacactgatttactcggcatcctaccggtacagtggagtccctgatcgcttcacaggcagtggatctgggacagatttcactctcaccatcagcaatgtgcagtctgaagacttggcagagtatttctgtcagcaatataacagctatccgtacacgttcggaggggggaccaagctggaaataaaacgggctgatgctgcaccaactgtatccatcttcccaccatccagtgagcagttaacatctggaggtgcctcagtcgtgtgcttcttgaacaacttctaccccaaagacatcaatgtcaagtggaagattgatggcagtgaacgacaaaatggcgtcctgaacagttggactgatcaggacagcaaagacagcacctacagcatgagcagcaccctcacgttgaccaaggacgagtatgaacgacataacagctatacctgtgaggccactcacaagacatcaacttcacccattgtcaagagcttcaacaggaatgagtgt

SEQ ID NO: 110 - protein, 214 aa, Artificial Sequence
  source: /note="Description of Artificial Sequence: Synthetic polypeptide"
DIVMTQSQKFMSTSVGDRVSVTCKASQNVGTNVAWYQQKLGQSPKTLIYSASYRYSGVPDRFTGSGSGTDFTLTISNVQSEDLAEYFCQQYNSYPYTFGGGTKLEIKRADAAPTVSIFPPSSEQLTSGGASVVCFLNNFYPKDINVKWKIDGSERQNGVLNSWTDQDSKDSTYSMSSTLTLTKDEYERHNSYTCEATHKTSTSPIVKSFNRNEC

SEQ ID NO: 111 - DNA, 1329 bp, Artificial Sequence
  source: /note="Description of Artificial Sequence: Synthetic polynucleotide"
caggttactctgaaagagtctggccctgggatattgcagccctcccagaccctcagtctgacttgttctttctctgggttttcactgaacacttatggtatgggtgtgagctggattcgtcagccttcaggaaagggtctggagtggctggcacacatttactgggatgatgacaagcgctataacccatccctgaagagccggctcacaatctccaaggatgcctccaacaaccgggtcttcctcaagatcaccagtgtggacactgcagatactgccacatactactgtgctcaaagaggttatgatgattactggggttactggggccaagggactctggtcactatctctgcagccaaaacgacacccccatctgtctatccactggcccctggatctgctgcccaaactaactccatggtgaccctgggatgcctggtcaagggctatttccctgagccagtgacagtgacctggaactctggatccctgtccagcggtgtgcacaccttcccagctgtcctgcagtctgacctctacactctgagcagctcagtgactgtcccctccagcacctggcccagcgagaccgtcacctgcaacgttgcccacccggccagcagcaccaaggtggacaagaaaattgtgcccagggattgtggttgtaagccttgcatatgtacagtcccagaagtatcatctgtcttcatcttccccccaaagcccaaggatgtgctcaccattactctgactcctaaggtcacgtgtgttgtggtagacatcagcaaggatgatcccgaggtccagttcagctggtttgtagatgatgtggaggtgcacacagctcagacgcaaccccgggaggagcagttcaacagcactttccgctcagtcagtgaacttcccatcatgcaccaggactggctcaatggcaaggagttcaaatgcagggtcaacagtgcagctttccctgcccccatcgagaaaaccatctccaaaaccaaaggcagaccgaaggctccacaggtgtacaccattccacctcccaaggagcagatggccaaggataaagtcagtctgacctgcatgataacagacttcttccctgaagacattactgtggagtggcagtggaatgggcagccagcggagaactacaagaacactcagcccatcatggacacagatggctcttacttcgtctacagcaagctcaatgtgcagaagagcaactgggaggcaggaaatactttcacctgctctgtgttacatgagggcctgcacaaccaccatactgagaagagcctctcccactctcctggtaaa

SEQ ID NO: 112 - protein, 443 aa, Artificial Sequence
  source: /note="Description of Artificial Sequence: Synthetic polypeptide"
QVTLKESGPGILQPSQTLSLTCSFSGFSLNTYGMGVSWIRQPSGKGLEWLAHIYWDDDKRYNPSLKSRLTISKDASNNRVFLKITSVDTADTATYYCAQRGYDDYWGYWGQGTLVTISAAKTTPPSVYPLAPGSAAQTNSMVTLGCLVKGYFPEPVTVTWNSGSLSSGVHTFPAVLQSDLYTLSSSVTVPSSTWPSETVTCNVAHPASSTKVDKKIVPRDCGCKPCICTVPEVSSVFIFPPKPKDVLTITLTPKVTCVVVDISKDDPEVQFSWFVDDVEVHTAQTQPREEQFNSTFRSVSELPIMHQDWLNGKEFKCRVNSAAFPAPIEKTISKTKGRPKAPQVYTIPPPKEQMAKDKVSLTCMITDFFPEDITVEWQWNGQPAENYKNTQPIMDTDGSYFVYSKLNVQKSNWEAGNTFTCSVLHEGLHNHHTEKSLSHSPGK

SEQ ID NO: 113 - DNA, 642 bp, Artificial Sequence
  source: /note="Description of Artificial Sequence: Synthetic polynucleotide"
gacattgtgatgacccagtctcaaaaattcatgtccacatcagtaggagacagggtcagcgtcacctgcaaggccagtcagaatgtgggtactaatgtagcctggtttcaacagaaaccaggtcaatctcctaaagcactgatttactcggcatcttaccggtacagtggagtccctgatcgcttcacaggcagtggatctgggacagatttcattctcaccatcagcaatgtgcagtctgaagacctggcagagtatttctgtcagcaatataacaactatcctctcacgttcggtgctgggaccaagctggagctgaaacgggctgatgctgcaccaactgtatccatcttcccaccatccagtgagcagttaacatctggaggtgcctcagtcgtgtgcttcttgaacaacttctaccccaaagacatcaatgtcaagtggaagattgatggcagtgaacgacaaaatggcgtcctgaacagttggactgatcaggacagcaaagacagcacctacagcatgagcagcaccctcacgttgaccaaggacgagtatgaacgacataacagctatacctgtgaggccactcacaagacatcaacttcacccattgtcaagagcttcaacaggaatgagtgt

SEQ ID NO: 114 - protein, 214 aa, Artificial Sequence
  source: /note="Description of Artificial Sequence: Synthetic polypeptide"
DIVMTQSQKFMSTSVGDRVSVTCKASQNVGTNVAWFQQKPGQSPKALIYSASYRYSGVPDRFTGSGSGTDFILTISNVQSEDLAEYFCQQYNNYPLTFGAGTKLELKRADAAPTVSIFPPSSEQLTSGGASVVCFLNNFYPKDINVKWKIDGSERQNGVLNSWTDQDSKDSTYSMSSTLTLTKDEYERHNSYTCEATHKTSTSPIVKSFNRNEC

SEQ ID NO: 115 - DNA, 1368 bp, Artificial Sequence
  source: /note="Description of Artificial Sequence: Synthetic polynucleotide"
gaggtcctgctgcaacagtctggacctgaggtggtgaagcctggggcttcagtgaagataccctgcaaggcttctggatacacattcactgactacaacatggactgggtgaagcagagccatggaaagagccttgagtggattggagagattaatcctaacaatggtggtactttctacaaccagaagttcaagggcaaggccacattgactgtagacaagtcctccagcacagcctacatggagctccgcagcctgacatctgaggacactgcagtctattactgtgcaagagaggcaattactacggtaggcgctatggactactggggtcaaggaacctcagtcaccgtctcctcagccaaaacaacacccccatcagtctatccactggcccctgggtgtggagatacaactggttcctccgtgactctgggatgcctggtcaagggctacttccctgagtcagtgactgtgacttggaactctggatccctgtccagcagtgtgcacaccttcccagctctcctgcagtctggactctacactatgagcagctcagtgactgtcccctccagcacctggccaagtcagaccgtcacctgcagcgttgctcacccagccagcagcaccacggtggacaaaaaacttgagcccagcgggcccatttcaacaatcaacccctgtcctccatgcaaggagtgtcacaaatgcccagctcctaacctcgagggtggaccatccgtcttcatcttccctccaaatatcaaggatgtactcatgatctccctgacacccaaggtcacgtgtgtggtggtggatgtgagcgaggatgacccagacgtccagatcagctggtttgtgaacaacgtggaagtacacacagctcagacacaaacccatagagaggattacaacagtactatccgggtggtcagcaccctccccatccagcaccaggactggatgagtggcaaggagttcaaatgcaaggtcaacaacaaagacctcccatcacccatcgagagaaccatctcaaaaattaaagggctagtcagagctccacaagtatacatcttgccgccaccagcagagcagttgtccaggaaagatgtcagtctcacttgcctggtcgtgggcttcaaccctggagacatcagtgtggagtggaccagcaatgggcatacagaggagaactacaaggacaccgcaccagtcctagactctgacggttcttacttcatatatagcaagctcaatatgaaaacaagcaagtgggagaaaacagattccttctcatgcaacgtgagacacgagggtctgaaaaattactacctgaagaagaccatctcccggtctccgggtaaa

SEQ ID NO: 116 - protein, 456 aa, Artificial Sequence
  source: /note="Description of Artificial Sequence: Synthetic polypeptide"
EVLLQQSGPEVVKPGASVKIPCKASGYTFTDYNMDWVKQSHGKSLEWIGEINPNNGGTFYNQKFKGKATLTVDKSSSTAYMELRSLTSEDTAVYYCAREAITTVGAMDYWGQGTSVTVSSAKTTPPSVYPLAPGCGDTTGSSVTLGCLVKGYFPESVTVTWNSGSLSSSVHTFPALLQSGLYTMSSSVTVPSSTWPSQTVTCSVAHPASSTTVDKKLEPSGPISTINPCPPCKECHKCPAPNLEGGPSVFIFPPNIKDVLMISLTPKVTCVVVDVSEDDPDVQISWFVNNVEVHTAQTQTHREDYNSTIRVVSTLPIQHQDWMSGKEFKCKVNNKDLPSPIERTISKIKGLVRAPQVYILPPPAEQLSRKDVSLTCLVVGFNPGDISVEWTSNGHTEENYKDTAPVLDSDGSYFIYSKLNMKTSKWEKTDSFSCNVRHEGLKNYYLKKTISRSPGK

SEQ ID NO: 117 - DNA, 642 bp, Artificial Sequence
  source: /note="Description of Artificial Sequence: Synthetic polynucleotide"
gacatccagatgactcagtctccagcctccctatctgcatctgtgggagaaactgtcaccatcacatgtcgagcaagtgggaatattcacaattatttagcatggtatcagcagaaacagggaaaatctcctcagctcctggtctataatgcaaaaaccttagcagatggtgtgccatcaaggttcagtggcagtggatcaggaacacaatattctctcaagatcaacagcctgcagcctgaagattttgggagttattactgtcaacatttttggagttctccttacacgttcggaggggggaccaagctggaaataaaacgggctgatgctgcaccaactgtatccatcttcccaccatccagtgagcagttaacatctggaggtgcctcagtcgtgtgcttcttgaacaacttctaccccaaagacatcaatgtcaagtggaagattgatggcagtgaacgacaaaatggcgtcctgaacagttggactgatcaggacagcaaagacagcacctacagcatgagcagcaccctcacgttgaccaaggacgagtatgaacgacataacagctatacctgtgaggccactcacaagacatcaacttcacccattgtcaagagcttcaacaggaatgagtgt

SEQ ID NO: 118 - protein, 214 aa, Artificial Sequence
  source: /note="Description of Artificial Sequence: Synthetic polypeptide"
DIQMTQSPASLSASVGETVTITCRASGNIHNYLAWYQQKQGKSPQLLVYNAKTLADGVPSRFSGSGSGTQYSLKINSLQPEDFGSYYCQHFWSSPYTFGGGTKLEIKRADAAPTVSIFPPSSEQLTSGGASVVCFLNNFYPKDINVKWKIDGSERQNGVLNSWTDQDSKDSTYSMSSTLTLTKDEYERHNSYTCEATHKTSTSPIVKSFNRNEC

SEQ ID NO: 119 - DNA, 1329 bp, Artificial Sequence
  source: /note="Description of Artificial Sequence: Synthetic polynucleotide"
caggttactctgaaagagtctggccctggaatattgcagccctcccagaccctcagtctgacttgttctttctctgggttttcactgagcacttatggtatgggtgtaggctggattcgtcagccttcaggaaagggtctagagtggctggcagacatttggtgggatgacgataagtactataacccatccctgaagagccggctcacaatctccaaggatacctccagcaatgaggtattcctcaagatcgccattgtggacactgcagatactgccacttactactgtgctcgaagaggtcactactctgctatggactactggggtcaaggaacctcagtcaccgtctcctcagccaaaacgacacccccatctgtctatccactggcccctggatctgctgcccaaactaactccatggtgaccctgggatgcctggtcaagggctatttccctgagccagtgacagtgacctggaactctggatccctgtccagcggtgtgcacaccttcccagctgtcctgcagtctgacctctacactctgagcagctcagtgactgtcccctccagcacctggcccagcgagaccgtcacctgcaacgttgcccacccggccagcagcaccaaggtggacaagaaaattgtgcccagggattgtggttgtaagccttgcatatgtacagtcccagaagtatcatctgtcttcatcttccccccaaagcccaaggatgtgctcaccattactctgactcctaaggtcacgtgtgttgtggtagacatcagcaaggatgatcccgaggtccagttcagctggtttgtagatgatgtggaggtgcacacagctcagacgcaaccccgggaggagcagttcaacagcactttccgctcagtcagtgaacttcccatcatgcaccaggactggctcaatggcaaggagttcaaatgcagggtcaacagtgcagctttccctgcccccatcgagaaaaccatctccaaaaccaaaggcagaccgaaggctccacaggtgtacaccattccacctcccaaggagcagatggccaaggataaagtcagtctgacctgcatgataacagacttcttccctgaagacattactgtggagtggcagtggaatgggcagccagcggagaactacaagaacactcagcccatcatggacacagatggctcttacttcgtctacagcaagctcaatgtgcagaagagcaactgggaggcaggaaatactttcacctgctctgtgttacatgagggcctgcacaaccaccatactgagaagagcctctcccactctcctggtaaa

SEQ ID NO: 120 - protein, 443 aa, Artificial Sequence
  source: /note="Description of Artificial Sequence: Synthetic polypeptide"
QVTLKESGPGILQPSQTLSLTCSFSGFSLSTYGMGVGWIRQPSGKGLEWLADIWWDDDKYYNPSLKSRLTISKDTSSNEVFLKIAIVDTADTATYYCARRGHYSAMDYWGQGTSVTVSSAKTTPPSVYPLAPGSAAQTNSMVTLGCLVKGYFPEPVTVTWNSGSLSSGVHTFPAVLQSDLYTLSSSVTVPSSTWPSETVTCNVAHPASSTKVDKKIVPRDCGCKPCICTVPEVSSVFIFPPKPKDVLTITLTPKVTCVVVDISKDDPEVQFSWFVDDVEVHTAQTQPREEQFNSTFRSVSELPIMHQDWLNGKEFKCRVNSAAFPAPIEKTISKTKGRPKAPQVYTIPPPKEQMAKDKVSLTCMITDFFPEDITVEWQWNGQPAENYKNTQPIMDTDGSYFVYSKLNVQKSNWEAGNTFTCSVLHEGLHNHHTEKSLSHSPGK

SEQ ID NO: 121 - DNA, 642 bp, Artificial Sequence
  source: /note="Description of Artificial Sequence: Synthetic polynucleotide"
gacattgtaatgacccagtctcaaaaattcatgtccacatcagtaggagacagggtcagcgtcacctgcaaggccagtcagaatgtgggtactaatgtagcctggtatcaacagaaaccagggcaatctcctaaagcactgatttactcgccatcctaccggtacagtggagtccctgatcgcttcacaggcagtggatctgggacagatttcactctcaccatcagcaatgtgcagtctgaagacttggcagaatatttctgtcagcaatataacagctatcctcacacgttcggaggggggaccaagctggaaatgaaacgggctgatgctgcaccaactgtatccatcttcccaccatccagtgagcagttaacatctggaggtgcctcagtcgtgtgcttcttgaacaacttctaccccaaagacatcaatgtcaagtggaagattgatggcagtgaacgacaaaatggcgtcctgaacagttggactgatcaggacagcaaagacagcacctacagcatgagcagcaccctcacgttgaccaaggacgagtatgaacgacataacagctatacctgtgaggccactcacaagacatcaacttcacccattgtcaagagcttcaacaggaatgagtgt

SEQ ID NO: 122 - protein, 214 aa, Artificial Sequence
  source: /note="Description of Artificial Sequence: Synthetic polypeptide"
DIVMTQSQKFMSTSVGDRVSVTCKASQNVGTNVAWYQQKPGQSPKALIYSPSYRYSGVPDRFTGSGSGTDFTLTISNVQSEDLAEYFCQQYNSYPHTFGGGTKLEMKRADAAPTVSIFPPSSEQLTSGGASVVCFLNNFYPKDINVKWKIDGSERQNGVLNSWTDQDSKDSTYSMSSTLTLTKDEYERHNSYTCEATHKTSTSPIVKSFNRNEC

SEQ ID NO: 123 - DNA, 1335 bp, Artificial Sequence
  source: /note="Description of Artificial Sequence: Synthetic polynucleotide"
caggttactctgaaagagtctggccctgggatattgcagccctcccagaccctcagtctgacttgttctttctctgggttttcactgagcacttctggtatgggtgtgagttggattcgtcagccttcaggaaagggtctggagtggctggcacacaatgactgggatgatgacaagcgctataagtcatccctgaagagccggctcacaatatccaaggatacctccagaaaccaggtattcctcaagatcaccagtgtggacactgcagatactgccacatactactgtgctcgaagagttgggggattagagggctattttgattactggggccaaggcaccactctcacagtctcctcagccaaaacgacacccccatctgtctatccactggcccctggatctgctgcccaaactaactccatggtgaccctgggatgcctggtcaagggctatttccctgagccagtgacagtgacctggaactctggatccctgtccagcggtgtgcacaccttcccagctgtcctgcagtctgacctctacactctgagcagctcagtgactgtcccctccagcacctggcccagcgagaccgtcacctgcaacgttgcccacccggccagcagcaccaaggtggacaagaaaattgtgcccagggattgtggttgtaagccttgcatatgtacagtcccagaagtatcatctgtcttcatcttccccccaaagcccaaggatgtgctcaccattactctgactcctaaggtcacgtgtgttgtggtagacatcagcaaggatgatcccgaggtccagttcagctggtttgtagatgatgtggaggtgcacacagctcagacgcaaccccgggaggagcagttcaacagcactttccgctcagtcagtgaacttcccatcatgcaccaggactggctcaatggcaaggagttcaaatgcagggtcaacagtgcagctttccctgcccccatcgagaaaaccatctccaaaaccaaaggcagaccgaaggctccacaggtgtacaccattccacctcccaaggagcagatggccaaggataaagtcagtctgacctgcatgataacagacttcttccctgaagacattactgtggagtggcagtggaatgggcagccagcggagaactacaagaacactcagcccatcatggacacagatggctcttacttcgtctacagcaagctcaatgtgcagaagagcaactgggaggcaggaaatactttcacctgctctgtgttacatgagggcctgcacaaccaccatactgagaagagcctctcccactctcctggtaaa

SEQ ID NO: 124 - protein, 445 aa, Artificial Sequence
  source: /note="Description of Artificial Sequence: Synthetic polypeptide"
QVTLKESGPGILQPSQTLSLTCSFSGFSLSTSGMGVSWIRQPSGKGLEWLAHNDWDDDKRYKSSLKSRLTISKDTSRNQVFLKITSVDTADTATYYCARRVGGLEGYFDYWGQGTTLTVSSAKTTPPSVYPLAPGSAAQTNSMVTLGCLVKGYFPEPVTVTWNSGSLSSGVHTFPAVLQSDLYTLSSSVTVPSSTWPSETVTCNVAHPASSTKVDKKIVPRDCGCKPCICTVPEVSSVFIFPPKPKDVLTITLTPKVTCVVVDISKDDPEVQFSWFVDDVEVHTAQTQPREEQFNSTFRSVSELPIMHQDWLNGKEFKCRVNSAAFPAPIEKTISKTKGRPKAPQVYTIPPPKEQMAKDKVSLTCMITDFFPEDITVEWQWNGQPAENYKNTQPIMDTDGSYFVYSKLNVQKSNWEAGNTFTCSVLHEGLHNHHTEKSLSHSPGK

SEQ ID NO: 125 - DNA, 654 bp, Artificial Sequence
  source: /note="Description of Artificial Sequence: Synthetic polynucleotide"
gacattgtgctgacacagtctcctgcttccttagctgtatctctggggcagagggccaccatctcatgcagggccagccaaagtgtcagtacatctaggtttagttatatgcactggttccaacagaaaccaggacaggcacccaaactcctcatcaagtatgcatccaacctagaatctggggtccctgccaggttcagtggcagtgggtctgggacagacttcaccctcaacatccatcctgtggagggggaggatactgcaacatattactgtcagcacagttgggagattccgtacacgttcggaggggggaccaagctggaaataaaacgggctgatgctgcaccaactgtatccatcttcccaccatccagtgagcagttaacatctggaggtgcctcagtcgtgtgcttcttgaacaacttctaccccaaagacatcaatgtcaagtggaagattgatggcagtgaacgacaaaatggcgtcctgaacagttggactgatcaggacagcaaagacagcacctacagcatgagcagcaccctcacgttgaccaaggacgagtatgaacgacataacagctatacctgtgaggccactcacaagacatcaacttcacccattgtcaagagcttcaacaggaatgagtgt

SEQ ID NO: 126 - protein, 218 aa, Artificial Sequence
  source: /note="Description of Artificial Sequence: Synthetic polypeptide"
DIVLTQSPASLAVSLGQRATISCRASQSVSTSRFSYMHWFQQKPGQAPKLLIKYASNLESGVPARFSGSGSGTDFTLNIHPVEGEDTATYYCQHSWEIPYTFGGGTKLEIKRADAAPTVSIFPPSSEQLTSGGASVVCFLNNFYPKDINVKWKIDGSERQNGVLNSWTDQDSKDSTYSMSSTLTLTKDEYERHNSYTCEATHKTSTSPIVKSFNRNEC

SEQ ID NO: 127 - DNA, 360 bp, Artificial Sequence
  source: /note="Description of Artificial Sequence: Synthetic polynucleotide"
gaagtgttgttgcagcagtcagggccggagttggtaaaaccgggagcgtcggtgaaaatcccgtgcaaagcgtcggggtatacgtttacggactataacatggattgggtgaaacagtcgcatgggaaatcgcttgaatggattggtcagatcaatccgaataatggaggaatcttctttaatcagaagtttaaaggaaaagcgacgcttacagtcgataagtcgtcgaacacggcgttcatggaagtacggtcgcttacgtcggaagatacggcggtctattactgtgcgagggaggcgattacgacggtgggagcgatggactattggggacaagggacgtcggtcacggtatcgtcg

SEQ ID NO: 128 - protein, 7 aa, Artificial Sequence
  source: /note="Description of Artificial Sequence: Synthetic peptide"
GYTFTSY

SEQ ID NO: 129 - DNA, 357 bp, Artificial Sequence
  source: /note="Description of Artificial Sequence: Synthetic polynucleotide"
caggtgacactcaaagaatcaggacccggaatccttcagcccagccagaccttgtcgctgacttgttcgttctccggtttcagcctgaatacttatgggatgggtgtgtcatggatcaggcaaccgtccgggaaaggattggagtggctcgcgcacatctactgggacgatgacaaacgctacaatccttcgctgaagagccgattgacgatttccaaggatgcctcgaacaaccgggtatttcttaagatcacgtcggtcgatacggcagacacggcgacctattactgcgcccaaagagggtacgatgactattggggatattggggccaggggacactcgtcacaatttcagct

SEQ ID NO: 130 - protein, 9 aa, Artificial Sequence
  source: /note="Description of Artificial Sequence: Synthetic peptide"
GFSLSTYGM

SEQ ID NO: 131 - DNA, 357 bp, Artificial Sequence
  source: /note="Description of Artificial Sequence: Synthetic polynucleotide"
caggtcacgctgaaagagtcaggtcccggaatccttcaaccttcgcagacattgtcactcacatgttccttctccgggttctcgctctcgacttatggcatgggtgtaggatggattcggcagcccagcgggaaggggcttgagtggttggcggatatctggtgggacgacgacaaatactacaatccgagcctgaagtcccgcctcaccatttcgaaagatacgtcatcaaacgaagtctttttgaagatcgccatcgtggacacggcggatacagcgacgtattactgcgccagaaggggacactacagcgcaatggattattggggacaggggacctcggtgactgtgtcgtcc

SEQ ID NO: 132 - protein, 9 aa, Artificial Sequence
  source: /note="Description of Artificial Sequence: Synthetic peptide"
GFSLNTYGM

SEQ ID NO: 133 - DNA, 321 bp, Artificial Sequence
  source: /note="Description of Artificial Sequence: Synthetic polynucleotide"
gacatccaaatgacccagtcacccgcgagcctttcggcgtcggtcggagaaacggtcacgatcacgtgccggacatcagagaatctccataactacctcgcgtggtatcaacagaagcaggggaagtcgccccagttgcttgtatacgatgcgaaaacgttggcggatggggtgccgtccagattctcgggatcgggctcggggacgcagtactcgctcaagatcaattcgctgcagccggaggactttgggtcgtactattgtcagcatttttggtcatcaccgtatacatttggaggtggaacgaaacttgagattaag

SEQ ID NO: 134 - protein, 9 aa, Artificial Sequence
  source: /note="Description of Artificial Sequence: Synthetic peptide"
GFSLSTSGM

SEQ ID NO: 135 - DNA, 321 bp, Artificial Sequence
  source: /note="Description of Artificial Sequence: Synthetic polynucleotide"
gatatcgtcatgacccagtcccagaagttcatgtcaacttcagtgggagacagagtgtccgtcacatgtaaagcctcgcaaaatgtgggaaccaacgtagcgtggttccagcagaaacctggccaatcaccgaaggcactgatctactcggccagctataggtactcgggagtaccagatcggtttacggggtcggggagcgggacggactttatcctcactatttccaatgtccagtcggaggaccttgcggaatacttctgccagcagtataacaactatcccctcacgtttggtgctggtacaaaattggagttgaag

SEQ ID NO: 136 - protein, 8 aa, Artificial Sequence
  source: /note="Description of Artificial Sequence: Synthetic peptide"
GYTFTDYN

SEQ ID NO: 137 - DNA, 321 bp, Artificial Sequence
  source: /note="Description of Artificial Sequence: Synthetic polynucleotide"
gacatcgtgatgacacagtcacagaaattcatgtccacatccgtcggtgatagagtatccgtcacgtgtaaggcctcgcaaaacgtaggaactaatgtggcgtggtatcaacagaagccaggacagtcacccaaagcactcatctacagcccctcatatcggtacagcggggtgccggacaggttcacgggatcggggagcgggaccgattttacactgaccatttcgaatgtccagtcggaggaccttgcggaatacttctgccagcagtataactcgtaccctcacacgtttggaggtggcactaagttggagatgaaa

SEQ ID NO: 138 - protein, 8 aa, Artificial Sequence
  source: /note="Description of Artificial Sequence: Synthetic peptide"
GYTFTSYW

SEQ ID NO: 139 - protein, 5 aa, Artificial Sequence
  source: /note="Description of Artificial Sequence: Synthetic peptide"
GGGGS

SEQ ID NO: 140 - protein, 10 aa, Artificial Sequence
  source: /note="Description of Artificial Sequence: Synthetic peptide"
GFSLSTYGMG

SEQ ID NO: 141 - protein, 10 aa, Artificial Sequence
  source: /note="Description of Artificial Sequence: Synthetic peptide"
GFSLNTYGMG

SEQ ID NO: 142 - protein, 10 aa, Artificial Sequence
  source: /note="Description of Artificial Sequence: Synthetic peptide"
GFSLSTSGMG

SEQ ID NO: 143 - protein, 6 aa, Artificial Sequence
  source: /note="Description of Artificial Sequence: Synthetic peptide"
NPNNGG

SEQ ID NO: 144 - protein, 6 aa, Artificial Sequence
  source: /note="Description of Artificial Sequence: Synthetic peptide"
NPSNGR

SEQ ID NO: 145 - protein, 5 aa, Artificial Sequence
  source: /note="Description of Artificial Sequence: Synthetic peptide"
YWDDD

SEQ ID NO: 146 - protein, 5 aa, Artificial Sequence
  source: /note="Description of Artificial Sequence: Synthetic peptide"
WWDDD

SEQ ID NO: 147 - protein, 5 aa, Artificial Sequence
  source: /note="Description of Artificial Sequence: Synthetic peptide"
DWDDD

SEQ ID NO: 148 - protein, 8 aa, Artificial Sequence
  source: /note="Description of Artificial Sequence: Synthetic peptide"
INPNNGGI

SEQ ID NO: 149 - protein, 8 aa, Artificial Sequence
  source: /note="Description of Artificial Sequence: Synthetic peptide"
INPSNGRS

SEQ ID NO: 150 - protein, 7 aa, Artificial Sequence
  source: /note="Description of Artificial Sequence: Synthetic peptide"
IYWDDDK

SEQ ID NO: 151 - protein, 8 aa, Artificial Sequence
  source: /note="Description of Artificial Sequence: Synthetic peptide"
INPNNGGT

SEQ ID NO: 152 - protein, 7 aa, Artificial Sequence
  source: /note="Description of Artificial Sequence: Synthetic peptide"
IWWDDDK

SEQ ID NO: 153 - protein, 7 aa, Artificial Sequence
  source: /note="Description of Artificial Sequence: Synthetic peptide"
NDWDDDK

SEQ ID NO: 154 - protein, 13 aa, Artificial Sequence
  source: /note="Description of Artificial Sequence: Synthetic peptide"
AREAITTVGAMDY

SEQ ID NO: 155 - protein, 11 aa, Artificial Sequence
  source: /note="Description of Artificial Sequence: Synthetic peptide"
AREVLDGAMDY

SEQ ID NO: 156 - protein, 11 aa, Artificial Sequence
  source: /note="Description of Artificial Sequence: Synthetic peptide"
AQTGYSNLFAY

SEQ ID NO: 157 - protein, 11 aa, Artificial Sequence
  source: /note="Description of Artificial Sequence: Synthetic peptide"
AQRGYDDYWGY

SEQ ID NO: 158 - protein, 11 aa, Artificial Sequence
  source: /note="Description of Artificial Sequence: Synthetic peptide"
ARRGHYSAMDY

SEQ ID NO: 159 - protein, 13 aa, Artificial Sequence
  source: /note="Description of Artificial Sequence: Synthetic peptide"
ARRVGGLEGYFDY

SEQ ID NO: 160 - protein, 6 aa, Artificial Sequence
  source: /note="Description of Artificial Sequence: Synthetic peptide"
ENLHNY

SEQ ID NO: 161 - protein, 10 aa, Artificial Sequence
  source: /note="Description of Artificial Sequence: Synthetic peptide"
ESVDNYGISF

SEQ ID NO: 162 - protein, 6 aa, Artificial Sequence
  source: /note="Description of Artificial Sequence: Synthetic peptide"
QNVGTN

SEQ ID NO: 163 - protein, 6 aa, Artificial Sequence
  source: /note="Description of Artificial Sequence: Synthetic peptide"
GNIHNY

SEQ ID NO: 164 - protein, 10 aa, Artificial Sequence
  source: /note="Description of Artificial Sequence: Synthetic peptide"
QSVSTSRFSY

SEQ ID NO: 165 - DNA, 972 bp, Mus sp.
gccaaaacgacacccccatctgtctatccactggcccctggatctgctgcccaaactaactccatggtgaccctgggatgcctggtcaagggctatttccctgagccagtgacagtgacctggaactctggatccctgtccagcggtgtgcacaccttcccagctgtcctgcagtctgacctctacactctgagcagctcagtgactgtcccctccagcacctggcccagcgagaccgtcacctgcaacgttgcccacccggccagcagcaccaaggtggacaagaaaattgtgcccagggattgtggttgtaagccttgcatatgtacagtcccagaagtatcatctgtcttcatcttccccccaaagcccaaggatgtgctcaccattactctgactcctaaggtcacgtgtgttgtggtagacatcagcaaggatgatcccgaggtccagttcagctggtttgtagatgatgtggaggtgcacacagctcagacgcaaccccgggaggagcagttcaacagcactttccgctcagtcagtgaacttcccatcatgcaccaggactggctcaatggcaaggagttcaaatgcagggtcaacagtgcagctttccctgcccccatcgagaaaaccatctccaaaaccaaaggcagaccgaaggctccacaggtgtacaccattccacctcccaaggagcagatggccaaggataaagtcagtctgacctgcatgataacagacttcttccctgaagacattactgtggagtggcagtggaatgggcagccagcggagaactacaagaacactcagcccatcatggacacagatggctcttacttcgtctacagcaagctcaatgtgcagaagagcaactgggaggcaggaaatactttcacctgctctgtgttacatgagggcctgcacaaccaccatactgagaagagcctctcccactctcctggtaaa

SEQ ID NO: 166 - protein, 324 aa, Mus sp.
AKTTPPSVYPLAPGSAAQTNSMVTLGCLVKGYFPEPVTVTWNSGSLSSGVHTFPAVLQSDLYTLSSSVTVPSSTWPSETVTCNVAHPASSTKVDKKIVPRDCGCKPCICTVPEVSSVFIFPPKPKDVLTITLTPKVTCVVVDISKDDPEVQFSWFVDDVEVHTAQTQPREEQFNSTFRSVSELPIMHQDWLNGKEFKCRVNSAAFPAPIEKTISKTKGRPKAPQVYTIPPPKEQMAKDKVSLTCMITDFFPEDITVEWQWNGQPAENYKNTQPIMDTDGSYFVYSKLNVQKSNWEAGNTFTCSVLHEGLHNHHTEKSLSHSPGK

SEQ ID NO: 167 - DNA, 1008 bp, Mus sp.
gccaaaacaacacccccatcagtctatccactggcccctgggtgtggagatacaactggttcctccgtgactctgggatgcctggtcaagggctacttccctgagtcagtgactgtgacttggaactctggatccctgtccagcagtgtgcacaccttcccagctctcctgcagtctggactctacactatgagcagctcagtgactgtcccctccagcacctggccaagtcagaccgtcacctgcagcgttgctcacccagccagcagcaccacggtggacaaaaaacttgagcccagcgggcccatttcaacaatcaacccctgtcctccatgcaaggagtgtcacaaatgcccagctcctaacctcgagggtggaccatccgtcttcatcttccctccaaatatcaaggatgtactcatgatctccctgacacccaaggtcacgtgtgtggtggtggatgtgagcgaggatgacccagacgtccagatcagctggtttgtgaacaacgtggaagtacacacagctcagacacaaacccatagagaggattacaacagtactatccgggtggtcagcaccctccccatccagcaccaggactggatgagtggcaaggagttcaaatgcaaggtcaacaacaaagacctcccatcacccatcgagagaaccatctcaaaaattaaagggctagtcagagctccacaagtatacatcttgccgccaccagcagagcagttgtccaggaaagatgtcagtctcacttgcctggtcgtgggcttcaaccctggagacatcagtgtggagtggaccagcaatgggcatacagaggagaactacaaggacaccgcaccagtcctagactctgacggttcttacttcatatatagcaagctcaatatgaaaacaagcaagtgggagaaaacagattccttctcatgcaacgtgagacacgagggtctgaaaaattactacctgaagaagaccatctcccggtctccgggtaaa

SEQ ID NO: 168 - protein, 336 aa, Mus sp.
AKTTPPSVYPLAPGCGDTTGSSVTLGCLVKGYFPESVTVTWNSGSLSSSVHTFPALLQSGLYTMSSSVTVPSSTWPSQTVTCSVAHPASSTTVDKKLEPSGPISTINPCPPCKECHKCPAPNLEGGPSVFIFPPNIKDVLMISLTPKVTCVVVDVSEDDPDVQISWFVNNVEVHTAQTQTHREDYNSTIRVVSTLPIQHQDWMSGKEFKCKVNNKDLPSPIERTISKIKGLVRAPQVYILPPPAEQLSRKDVSLTCLVVGFNPGDISVEWTSNGHTEENYKDTAPVLDSDGSYFIYSKLNMKTSKWEKTDSFSCNVRHEGLKNYYLKKTISRSPGK

SEQ ID NO: 169 - DNA, 321 bp, Mus sp.
cgggctgatgctgcaccaactgtatccatcttcccaccatccagtgagcagttaacatctggaggtgcctcagtcgtgtgcttcttgaacaacttctaccccaaagacatcaatgtcaagtggaagattgatggcagtgaacgacaaaatggcgtcctgaacagttggactgatcaggacagcaaagacagcacctacagcatgagcagcaccctcacgttgaccaaggacgagtatgaacgacataacagctatacctgtgaggccactcacaagacatcaacttcacccattgtcaagagcttcaacaggaatgagtgt

SEQ ID NO: 170 - protein, 107 aa, Mus sp.
RADAAPTVSIFPPSSEQLTSGGASVVCFLNNFYPKDINVKWKIDGSERQNGVLNSWTDQDSKDSTYSMSSTLTLTKDEYERHNSYTCEATHKTSTSPIVKSFNRNEC

SEQ ID NO: 171 - DNA, 990 bp, Homo sapiens
gcctcaacaaaaggaccaagtgtgttcccactcgcccctagcagcaagagtacatccgggggcactgcagcactcggctgcctcgtcaaggattattttccagagccagtaaccgtgagctggaacagtggagcactcacttctggtgtccatacttttcctgctgtcctgcaaagctctggcctgtactcactcagctccgtcgtgaccgtgccatcttcatctctgggcactcagacctacatctgtaatgtaaaccacaagcctagcaatactaaggtcgataagcgggtggaacccaagagctgcgacaagactcacacttgtcccccatgccctgcccctgaacttctgggcggtcccagcgtctttttgttcccaccaaagcctaaagatactctgatgataagtagaacacccgaggtgacatgtgttgttgtagacgtttcccacgaggacccagaggttaagttcaactggtacgttgatggagtcgaagtacataatgctaagaccaagcctagagaggagcagtataatagtacataccgtgtagtcagtgttctcacagtgctgcaccaagactggctcaacggcaaagaatacaaatgcaaagtgtccaacaaagcactcccagcccctatcgagaagactattagtaaggcaaaggggcagcctcgtgaaccacaggtgtacactctgccacccagtagagaggaaatgacaaagaaccaagtctcattgacctgcctggtgaaaggcttctaccccagcgacatcgccgttgagtgggagagtaacggtcagcctgagaacaattacaagacaacccccccagtgctggatagtgacgggtctttctttctgtacagtaagctgactgtggacaagtcccgctggcagcagggtaacgtcttcagctgttccgtgatgcacgaggcattgcacaaccactacacccagaagtcactgagcctgagcccagggaag

SEQ ID NO: 172 - protein, 330 aa, Homo sapiens
ASTKGPSVFPLAPSSKSTSGGTAALGCLVKDYFPEPVTVSWNSGALTSGVHTFPAVLQSSGLYSLSSVVTVPSSSLGTQTYICNVNHKPSNTKVDKRVEPKSCDKTHTCPPCPAPELLGGPSVFLFPPKPKDTLMISRTPEVTCVVVDVSHEDPEVKFNWYVDGVEVHNAKTKPREEQYNSTYRVVSVLTVLHQDWLNGKEYKCKVSNKALPAPIEKTISKAKGQPREPQVYTLPPSREEMTKNQVSLTCLVKGFYPSDIAVEWESNGQPENNYKTTPPVLDSDGSFFLYSKLTVDKSRWQQGNVFSCSVMHEALHNHYTQKSLSLSPGK

SEQ ID NO: 173 - DNA, 321 bp, Homo sapiens
cgcacagttgctgcccccagcgtgttcattttcccacctagcgatgagcagctgaaaagcggtactgcctctgtcgtatgcttgctcaacaacttttacccacgtgaggctaaggtgcagtggaaagtggataatgcacttcaatctggaaacagtcaagagtccgtgacagaacaggacagcaaagactcaacttattcactctcttccaccctgactctgtccaaggcagactatgaaaaacacaaggtatacgcctgcgaggttacacaccagggtttgtctagtcctgtcaccaagtccttcaataggggcgaatgt

SEQ ID NO: 174 - protein, 107 aa, Homo sapiens [sequence omitted]

SEQ ID NO: 175 - DNA, 1350 bp, Artificial Sequence
  source: /note="Description of Artificial Sequence: Synthetic polynucleotide"
gaagtgttgttgcagcagtcagggccggagttggtaaaaccgggagcgtcggtgaaaatcccgtgcaaagcgtcggggtatacgtttacggactataacatggattgggtgaaacagtcgcatgggaaatcgcttgaatggattggtcagatcaatccgaataatggaggaatcttctttaatcagaagtttaaaggaaaagcgacgcttacagtcgataagtcgtcgaacacggcgttcatggaagtacggtcgcttacgtcggaagatacggcggtctattactgtgcgagggaggcgattacgacggtgggagcgatggactattggggacaagggacgtcggtcacggtatcgtcggcctcaacaaaaggaccaagtgtgttcccactcgcccctagcagcaagagtacatccgggggcactgcagcactcggctgcctcgtcaaggattattttccagagccagtaaccgtgagctggaacagtggagcactcacttctggtgtccatacttttcctgctgtcctgcaaagctctggcctgtactcactcagctccgtcgtgaccgtgccatcttcatctctgggcactcagacctacatctgtaatgtaaaccacaagcctagcaatactaaggtcgataagcgggtggaacccaagagctgcgacaagactcacacttgtcccccatgccctgcccctgaacttctgggcggtcccagcgtctttttgttcccaccaaagcctaaagatactctgatgataagtagaacacccgaggtgacatgtgttgttgtagacgtttcccacgaggacccagaggttaagttcaactggtacgttgatggagtcgaagtacataatgctaagaccaagcctagagaggagcagtataatagtacataccgtgtagtcagtgttctcacagtgctgcaccaagactggctcaacggcaaagaatacaaatgcaaagtgtccaacaaagcactcccagcccctatcgagaagactattagtaaggcaaaggggcagcctcgtgaaccacaggtgtacactctgccacccagtagagaggaaatgacaaagaaccaagtctcattgacctgcctggtgaaaggcttctaccccagcgacatcgccgttgagtgggagagtaacggtcagcctgagaacaattacaagacaacccccccagtgctggatagtgacgggtctttctttctgtacagtaagctgactgtggacaagtcccgctggcagcagggtaacgtcttcagctgttccgtgatgcacgaggcattgcacaaccactacacccagaagtcactgagcctgagcccagggaag

SEQ ID NO: 176 - protein, 450 aa, Artificial Sequence
  source: /note="Description of Artificial Sequence: Synthetic polypeptide"
EVLLQQSGPELVKPGASVKIPCKASGYTFTDYNMDWVKQSHGKSLEWIGQINPNNGGIFFNQKFKGKATLTVDKSSNTAFMEVRSLTSEDTAVYYCAREAITTVGAMDYWGQGTSVTVSSASTKGPSVFPLAPSSKSTSGGTAALGCLVKDYFPEPVTVSWNSGALTSGVHTFPAVLQSSGLYSLSSVVTVPSSSLGTQTYICNVNHKPSNTKVDKRVEPKSCDKTHTCPPCPAPELLGGPSVFLFPPKPKDTLMISRTPEVTCVVVDVSHEDPEVKFNWYVDGVEVHNAKTKPREEQYNSTYRVVSVLTVLHQDWLNGKEYKCKVSNKALPAPIEKTISKAKGQPREPQVYTLPPSREEMTKNQVSLTCLVKGFYPSDIAVEWESNGQPENNYKTTPPVLDSDGSFFLYSKLTVDKSRWQQGNVFSCSVMHEALHNHYTQKSLSLSPGK

SEQ ID NO: 177 - DNA, 1350 bp, Artificial Sequence
  source: /note="Description of Artificial Sequence: Synthetic polynucleotide"
caagtgcaacttgtgcagtcgggtgcggaagtcaaaaagccgggagcgtcggtgaaagtatcgtgtaaagcgtcgggatatacgtttacggactataacatggactgggtacgacaggcaccggggaaatcgttggaatggatcggacagattaatccgaacaatgggggaattttctttaatcagaaattcaaaggacgggcgacgttgacggtcgatacatcgacgaatacggcgtatatggaattgaggtcgcttcgctcggacgatacggcggtctattactgcgccagggaggcgatcacgacggtaggggcgatggattattggggacaggggacgcttgtgacggtatcgtcggcctcaacaaaaggaccaagtgtgttcccactcgcccctagcagcaagagtacatccgggggcactgcagcactcggctgcctcgtcaaggattattttccagagccagtaaccgtgagctggaacagtggagcactcacttctggtgtccatacttttcctgctgtcctgcaaagctctggcctgtactcactcagctccgtcgtgaccgtgccatcttcatctctgggcactcagacctacatctgtaatgtaaaccacaagcctagcaatactaaggtcgataagcgggtggaacccaagagctgcgacaagactcacacttgtcccccatgccctgcccctgaacttctgggcggtcccagcgtctttttgttcccaccaaagcctaaagatactctgatgataagtagaacacccgaggtgacatgtgttgttgtagacgtttcccacgaggacccagaggttaagttcaactggtacgttgatggagtcgaagtacataatgctaagaccaagcctagagaggagcagtataatagtacataccgtgtagtcagtgttctcacagtgctgcaccaagactggctcaacggcaaagaatacaaatgcaaagtgtccaacaaagcactcccagcccctatcgagaagactattagtaaggcaaaggggcagcctcgtgaaccacaggtgtacactctgccacccagtagagaggaaatgacaaagaaccaagtctcattgacctgcctggtgaaaggcttctaccccagcgacatcgccgttgagtgggagagtaacggtcagcctgagaacaattacaagacaacccccccagtgctggatagtgacgggtctttctttctgtacagtaagctgactgtggacaagtcccgctggcagcagggtaacgtcttcagctgttccgtgatgcacgaggcattgcacaaccactacacccagaagtcactgagcctgagcccagggaag

SEQ ID NO: 178 - protein, 450 aa, Artificial Sequence
  source: /note="Description of Artificial Sequence: Synthetic polypeptide"
QVQLVQSGAEVKKPGASVKVSCKASGYTFTDYNMDWVRQAPGKSLEWIGQINPNNGGIFFNQKFKGRATLTVDTSTNTAYMELRSLRSDDTAVYYCAREAITTVGAMDYWGQGTLVTVSSASTKGPSVFPLAPSSKSTSGGTAALGCLVKDYFPEPVTVSWNSGALTSGVHTFPAVLQSSGLYSLSSVVTVPSSSLGTQTYICNVNHKPSNTKVDKRVEPKSCDKTHTCPPCPAPELLGGPSVFLFPPKPKDTLMISRTPEVTCVVVDVSHEDPEVKFNWYVDGVEVHNAKTKPREEQYNSTYRVVSVLTVLHQDWLNGKEYKCKVSNKALPAPIEKTISKAKGQPREPQVYTLPPSREEMTKNQVSLTCLVKGFYPSDIAVEWESNGQPENNYKTTPPVLDSDGSFFLYSKLTVDKSRWQQGNVFSCSVMHEALHNHYTQKSLSLSPGK

SEQ ID NO: 179 - DNA, 1350 bp, Artificial Sequence
  source: /note="Description of Artificial Sequence: Synthetic polynucleotide"
caagtccagcttgtccagtcgggagcggaagtgaagaaaccggggtcgtcggtcaaagtatcgtgtaaagcgtcgggatatacgtttacggactataacatggattgggtacgacaggctccgggaaaatcattggaatggattggacagattaatccgaataatgggggtatcttctttaatcaaaagtttaaagggagggcgacgttgacggtggacaaatcgacaaatacggcgtatatggaattgtcgtcgcttcggtcggaggacacggcggtgtattactgcgcgagggaggcgatcacgacggtcggggcgatggattattggggacagggaacgcttgtgacggtatcgtcggcctcaacaaaaggaccaagtgtgttcccactcgcccctagcagcaagagtacatccgggggcactgcagcactcggctgcctcgtcaaggattattttccagagccagtaaccgtgagctggaacagtggagcactcacttctggtgtccatacttttcctgctgtcctgcaaagctctggcctgtactcactcagctccgtcgtgaccgtgccatcttcatctctgggcactcagacctacatctgtaatgtaaaccacaagcctagcaatactaaggtcgataagcgggtggaacccaagagctgcgacaagactcacacttgtcccccatgccctgcccctgaacttctgggcggtcccagcgtctttttgttcccaccaaagcctaaagatactctgatgataagtagaacacccgaggtgacatgtgttgttgtagacgtttcccacgaggacccagaggttaagttcaactggtacgttgatggagtcgaagtacataatgctaagaccaagcctagagaggagcagtataatagtacataccgtgtagtcagtgttctcacagtgctgcaccaagactggctcaacggcaaagaatacaaatgcaaagtgtccaacaaagcactcccagcccctatcgagaagactattagtaaggcaaaggggcagcctcgtgaaccacaggtgtacactctgccacccagtagagaggaaatgacaaagaaccaagtctcattgacctgcctggtgaaaggcttctaccccagcgacatcgccgttgagtgggagagtaacggtcagcctgagaacaattacaagacaacccccccagtgctggatagtgacgggtctttctttctgtacagtaagctgactgtggacaagtcccgctggcagcagggtaacgtcttcagctgttccgtgatgcacgaggcattgcacaaccactacacccagaagtcactgagcctgagcccagggaag

SEQ ID NO: 180 - protein, 450 aa, Artificial Sequence
  source: /note="Description of Artificial Sequence: Synthetic polypeptide"
QVQLVQSGAEVKKPGSSVKVSCKASGYTFTDYNMDWVRQAPGKSLEWIGQINPNNGGIFFNQKFKGRATLTVDKSTNTAYMELSSLRSEDTAVYYCAREAITTVGAMDYWGQGTLVTVSSASTKGPSVFPLAPSSKSTSGGTAALGCLVKDYFPEPVTVSWNSGALTSGVHTFPAVLQSSGLYSLSSVVTVPSSSLGTQTYICNVNHKPSNTKVDKRVEPKSCDKTHTCPPCPAPELLGGPSVFLFPPKPKDTLMISRTPEVTCVVVDVSHEDPEVKFNWYVDGVEVHNAKTKPREEQYNSTYRVVSVLTVLHQDWLNGKEYKCKVSNKALPAPIEKTISKAKGQPREPQVYTLPPSREEMTKNQVSLTCLVKGFYPSDIAVEWESNGQPENNYKTTPPVLDSDGSFFLYSKLTVDKSRWQQGNVFSCSVMHEALHNHYTQKSLSLSPGK

SEQ ID NO: 181 - DNA, 1350 bp, Artificial Sequence
  source: /note="Description of Artificial Sequence: Synthetic polynucleotide"
caggtccagcttgtgcaatcgggagcggaagtgaagaaaccgggagcgtcggtaaaagtctcgtgcaaagcgtcggggtatacgtttacggactataacatggactgggtgcgccaagcgcctggacagggtcttgaatggatggggcagattaatccgaataatggagggatcttctttaatcagaaattcaaaggaagggtaacgctgacgacagacacgtcaacatcgacggcctatatggaattgcggtcgttgcgatcagatgatacggcggtctactattgtgcgagggaggcgattacgacggtgggagcgatggattattggggacaggggacgttggtaacggtatcgtcggcctcaacaaaaggaccaagtgtgttcccactcgcccctagcagcaagagtacatccgggggcactgcagcactcggctgcctcgtcaaggattattttccagagccagtaaccgtgagctggaacagtggagcactcacttctggtgtccatacttttcctgctgtcctgcaaagctctggcctgtactcactcagctccgtcgtgaccgtgccatcttcatctctgggcactcagacctacatctgtaatgtaaaccacaagcctagcaatactaaggtcgataagcgggtggaacccaagagctgcgacaagactcacacttgtcccccatgccctgcccctgaacttctgggcggtcccagcgtctttttgttcccaccaaagcctaaagatactctgatgataagtagaacacccgaggtgacatgtgttgttgtagacgtttcccacgaggacccagaggttaagttcaactggtacgttgatggagtcgaagtacataatgctaagaccaagcctagagaggagcagtataatagtacataccgtgtagtcagtgttctcacagtgctgcaccaagactggctcaacggcaaagaatacaaatgcaaagtgtccaacaaagcactcccagcccctatcgagaagactattagtaaggcaaaggggcagcctcgtgaaccacaggtgtacactctgccacccagtagagaggaaatgacaaagaaccaagtctcattgacctgcctggtgaaaggcttctaccccagcgacatcgccgttgagtgggagagtaacggtcagcctgagaacaattacaagacaacccccccagtgctggatagtgacgggtctttctttctgtacagtaagctgactgtggacaagtcccgctggcagcagggtaacgtcttcagctgttccgtgatgcacgaggcattgcacaaccactacacccagaagtcactgagcctgagcccagggaag

SEQ ID NO: 182 - protein, 450 aa, Artificial Sequence
  source: /note="Description of Artificial Sequence: Synthetic polypeptide"
QVQLVQSGAEVKKPGASVKVSCKASGYTFTDYNMDWVRQAPGQGLEWMGQINPNNGGIFFNQKFKGRVTLTTDTSTSTAYMELRSLRSDDTAVYYCAREAITTVGAMDYWGQGTLVTVSSASTKGPSVFPLAPSSKSTSGGTAALGCLVKDYFPEPVTVSWNSGALTSGVHTFPAVLQSSGLYSLSSVVTVPSSSLGTQTYICNVNHKPSNTKVDKRVEPKSCDKTHTCPPCPAPELLGGPSVFLFPPKPKDTLMISRTPEVTCVVVDVSHEDPEVKFNWYVDGVEVHNAKTKPREEQYNSTYRVVSVLTVLHQDWLNGKEYKCKVSNKALPAPIEKTISKAKGQPREPQVYTLPPSREEMTKNQVSLTCLVKGFYPSDIAVEWESNGQPENNYKTTPPVLDSDGSFFLYSKLTVDKSRWQQGNVFSCSVMHEALHNHYTQKSLSLSPGK

SEQ ID NO: 183 - DNA, 1350 bp, Artificial Sequence
  source: /note="Description of Artificial Sequence: Synthetic polynucleotide"
caggtccagcttgtgcaatcgggagcggaagtgaagaaaccgggagcgtcggtaaaagtctcgtgcaaagcgtcggggtatacgtttacggactataacatggactgggtgcgccaagcgcctggacagagccttgaatggatggggcagattaatccgaataatggagggatcttctttaatcagaaattccagggaagggtaacgctgacgacagacacgtcaacatcgacggcctatatggaattgcggtcgttgcgatcagatgatacggcggtctactattgtgcgagggaggcgattacgacggtgggagcgatggattattggggacaggggacgttggtaacggtatcgtcggcctcaacaaaaggaccaagtgtgttcccactcgcccctagcagcaagagtacatccgggggcactgcagcactcggctgcctcgtcaaggattattttccagagccagtaaccgtgagctggaacagtggagcactcacttctggtgtccatacttttcctgctgtcctgcaaagctctggcctgtactcactcagctccgtcgtgaccgtgccatcttcatctctgggcactcagacctacatctgtaatgtaaaccacaagcctagcaatactaaggtcgataagcgggtggaacccaagagctgcgacaagactcacacttgtcccccatgccctgcccctgaacttctgggcggtcccagcgtctttttgttcccaccaaagcctaaagatactctgatgataagtagaacacccgaggtgacatgtgttgttgtagacgtttcccacgaggacccagaggttaagttcaactggtacgttgatggagtcgaagtacataatgctaagaccaagcctagagaggagcagtataatagtacataccgtgtagtcagtgttctcacagtgctgcaccaagactggctcaacggcaaagaatacaaatgcaaagtgtccaacaaagcactcccagcccctatcgagaagactattagtaaggcaaaggggcagcctcgtgaaccacaggtgtacactctgccacccagtagagaggaaatgacaaagaaccaagtctcattgacctgcctggtgaaaggcttctaccccagcgacatcgccgttgagtgggagagtaacggtcagcctgagaacaattacaagacaacccccccagtgctggatagtgacgggtctttctttctgtacagtaagctgactgtggacaagtcccgctggcagcagggtaacgtcttcagctgttccgtgatgcacgaggcattgcacaaccactacacccagaagtcactgagcctgagcccagggaag

SEQ ID NO: 184 - protein, 450 aa, Artificial Sequence
  source: /note="Description of Artificial Sequence: Synthetic polypeptide"
QVQLVQSGAEVKKPGASVKVSCKASGYTFTDYNMDWVRQAPGQSLEWMGQINPNNGGIFFNQKFQGRVTLTTDTSTSTAYMELRSLRSDDTAVYYCAREAITTVGAMDYWGQGTLVTVSSASTKGPSVFPLAPSSKSTSGGTAALGCLVKDYFPEPVTVSWNSGALTSGVHTFPAVLQSSGLYSLSSVVTVPSSSLGTQTYICNVNHKPSNTKVDKRVEPKSCDKTHTCPPCPAPELLGGPSVFLFPPKPKDTLMISRTPEVTCVVVDVSHEDPEVKFNWYVDGVEVHNAKTKPREEQYNSTYRVVSVLTVLHQDWLNGKEYKCKVSNKALPAPIEKTISKAKGQPREPQVYTLPPSREEMTKNQVSLTCLVKGFYPSDIAVEWESNGQPENNYKTTPPVLDSDGSFFLYSKLTVDKSRWQQGNVFSCSVMHEALHNHYTQKSLSLSPGK

SEQ ID NO: 185 - DNA, 1350 bp, Artificial Sequence
  source: /note="Description of Artificial Sequence: Synthetic polynucleotide"
caggtccagcttgtgcaatcgggagcggaagtgaagaaaccgggagcgtcggtaaaagtctcgtgcaaagcgtcggggtatacgtttacggactataacatggactgggtgcgccaagcgcctggacagggtcttgaatggatggggcagattaatccgaataatggagggatcttctttaatcagaaattccagggaagggtaacgctgacgacagacacgtcaacatcgacggcctatatggaattgcggtcgttgcgatcagatgatacggcggtctactattgtgcgagggaggcgattacgacggtgggagcgatggattattggggacaggggacgttggtaacggtatcgtcggcctcaacaaaaggaccaagtgtgttcccactcgcccctagcagcaagagtacatccgggggcactgcagcactcggctgcctcgtcaaggattattttccagagccagtaaccgtgagctggaacagtggagcactcacttctggtgtccatacttttcctgctgtcctgcaaagctctggcctgtactcactcagctccgtcgtgaccgtgccatcttcatctctgggcactcagacctacatctgtaatgtaaaccacaagcctagcaatactaaggtcgataagcgggtggaacccaagagctgcgacaagactcacacttgtcccccatgccctgcccctgaacttctgggcggtcccagcgtctttttgttcccaccaaagcctaaagatactctgatgataagtagaacacccgaggtgacatgtgttgttgtagacgtttcccacgaggacccagaggttaagttcaactggtacgttgatggagtcgaagtacataatgctaagaccaagcctagagaggagcagtataatagtacataccgtgtagtcagtgttctcacagtgctgcaccaagactggctcaacggcaaagaatacaaatgcaaagtgtccaacaaagcactcccagcccctatcgagaagactattagtaaggcaaaggggcagcctcgtgaaccacaggtgtacactctgccacccagtagagaggaaatgacaaagaaccaagtctcattgacctgcctggtgaaaggcttctaccccagcgacatcgccgttgagtgggagagtaacggtcagcctgagaacaattacaagacaacccccccagtgctggatagtgacgggtctttctttctgtacagtaagctgactgtggacaagtcccgctggcagcagggtaacgtcttcagctgttccgtgatgcacgaggcattgcacaaccactacacccagaagtcactgagcctgagcccagggaag

SEQ ID NO: 186 - protein, 450 aa, Artificial Sequence
  source: /note="Description of Artificial Sequence: Synthetic polypeptide"
QVQLVQSGAEVKKPGASVKVSCKASGYTFTDYNMDWVRQAPGQGLEWMGQINPNNGGIFFNQKFQGRVTLTTDTSTSTAYMELRSLRSDDTAVYYCAREAITTVGAMDYWGQGTLVTVSSASTKGPSVFPLAPSSKSTSGGTAALGCLVKDYFPEPVTVSWNSGALTSGVHTFPAVLQSSGLYSLSSVVTVPSSSLGTQTYICNVNHKPSNTKVDKRVEPKSCDKTHTCPPCPAPELLGGPSVFLFPPKPKDTLMISRTPEVTCVVVDVSHEDPEVKFNWYVDGVEVHNAKTKPREEQYNSTYRVVSVLTVLHQDWLNGKEYKCKVSNKALPAPIEKTISKAKGQPREPQVYTLPPSREEMTKNQVSLTCLVKGFYPSDIAVEWESNGQPENNYKTTPPVLDSDGSFFLYSKLTVDKSRWQQGNVFSCSVMHEALHNHYTQKSLSLSPGK

SEQ ID NO: 187 - DNA, 1350 bp, Artificial Sequence
  source: /note="Description of Artificial Sequence: Synthetic polynucleotide"
caagtacagcttgtacagtcgggagcggaagtcaagaaaccgggatcgtcggtcaaagtgtcgtgtaaagcgtcgggatatacgtttagcgactataacatggattgggtgcgacaagcgcctgggcagggacttgaatggatgggtcagatcaatccgaataatgggggaatctttttcaatcagaagtttaaagggagggtaacgctgacggcggataaaagcacgtcaacggcgtatatggagttgtcgtcgttgcggtcggaggacacggcggtctattactgcgcgagggaagcgattacgacggtgggagcgatggattattgggggcagggaacgcttgtaacggtgtcatcggcctcaacaaaaggaccaagtgtgttcccactcgcccctagcagcaagagtacatccgggggcactgcagcactcggctgcctcgtcaaggattattttccagagccagtaaccgtgagctggaacagtggagcactcacttctggtgtccatacttttcctgctgtcctgcaaagctctggcctgtactcactcagctccgtcgtgaccgtgccatcttcatctctgggcactcagacctacatctgtaatgtaaaccacaagcctagcaatactaaggtcgataagcgggtggaacccaagagctgcgacaagactcacacttgtcccccatgccctgcccctgaacttctgggcggtcccagcgtctttttgttcccaccaaagcctaaagatactctgatgataagtagaacacccgaggtgacatgtgttgttgtagacgtttcccacgaggacccagaggttaagttcaactggtacgttgatggagtcgaagtacataatgctaagaccaagcctagagaggagcagtataatagtacataccgtgtagtcagtgttctcacagtgctgcaccaagactggctcaacggcaaagaatacaaatgcaaagtgtccaacaaagcactcccagcccctatcgagaagactattagtaaggcaaaggggcagcctcgtgaaccacaggtgtacactctgccacccagtagagaggaaatgacaaagaaccaagtctcattgacctgcctggtgaaaggcttctaccccagcgacatcgccgttgagtgggagagtaacggtcagcctgagaacaattacaagacaacccccccagtgctggatagtgacgggtctttctttctgtacagtaagctgactgtggacaagtcccgctggcagcagggtaacgtcttcagctgttccgtgatgcacgaggcattgcacaaccactacacccagaagtcactgagcctgagcccagggaag

SEQ ID NO: 188 - protein, 450 aa, Artificial Sequence
  source: /note="Description of Artificial Sequence: Synthetic polypeptide"
QVQLVQSGAEVKKPGSSVKVSCKASGYTFSDYNMDWVRQAPGQGLEWMGQINPNNGGIFFNQKFKGRVTLTADKSTSTAYMELSSLRSEDTAVYYCAREAITTVGAMDYWGQGTLVTVSSASTKGPSVFPLAPSSKSTSGGTAALGCLVKDYFPEPVTVSWNSGALTSGVHTFPAVLQSSGLYSLSSVVTVPSSSLGTQTYICNVNHKPSNTKVDKRVEPKSCDKTHTCPPCPAPELLGGPSVFLFPPKPKDTLMISRTPEVTCVVVDVSHEDPEVKFNWYVDGVEVHNAKTKPREEQYNSTYRVVSVLTVLHQDWLNGKEYKCKVSNKALPAPIEKTISKAKGQPREPQVYTLPPSREEMTKNQVSLTCLVKGFYPSDIAVEWESNGQPENNYKTTPPVLDSDGSFFLYSKLTVDKSRWQQGNVFSCSVMHEALHNHYTQKSLSLSPGK

SEQ ID NO: 189 - DNA, 1350 bp, Artificial Sequence
  source: /note="Description of Artificial Sequence: Synthetic polynucleotide"
caagtacagcttgtacagtcgggagcggaagtcaagaaaccgggatcgtcggtcaaagtgtcgtgtaaagcgtcgggatatacgtttagcgactataacatggattgggtgcgacaagcgcctgggcagggacttgaatggatgggtcagatcaatccgaataatgggggaatctttttcaatcagaagtttcaggggagggtaacgctgacggcggataaaagcacgtcaacggcgtatatggagttgtcgtcgttgcggtcggaggacacggcggtctattactgcgcgagggaagcgattacgacggtgggagcgatggattattgggggcagggaacgcttgtaacggtgtcatcggcctcaacaaaaggaccaagtgtgttcccactcgcccctagcagcaagagtacatccgggggcactgcagcactcggctgcctcgtcaaggattattttccagagccagtaaccgtgagctggaacagtggagcactcacttctggtgtccatacttttcctgctgtcctgcaaagctctggcctgtactcactcagctccgtcgtgaccgtgccatcttcatctctgggcactcagacctacatctgtaatgtaaaccacaagcctagcaatactaaggtcgataagcgggtggaacccaagagctgcgacaagactcacacttgtcccccatgccctgcccctgaacttctgggcggtcccagcgtctttttgttcccaccaaagcctaaagatactctgatgataagtagaacacccgaggtgacatgtgttgttgtagacgtttcccacgaggacccagaggttaagttcaactggtacgttgatggagtcgaagtacataatgctaagaccaagcctagagaggagcagtataatagtacataccgtgtagtcagtgttctcacagtgctgcaccaagactggctcaacggcaaagaatacaaatgcaaagtgtccaacaaagcactcccagcccctatcgagaagactattagtaaggcaaaggggcagcctcgtgaaccacaggtgtacactctgccacccagtagagaggaaatgacaaagaaccaagtctcattgacctgcctggtgaaaggcttctaccccagcgacatcgccgttgagtgggagagtaacggtcagcctgagaacaattacaagacaacccccccagtgctggatagtgacgggtctttctttctgtacagtaagctgactgtggacaagtcccgctggcagcagggtaacgtcttcagctgttccgtgatgcacgaggcattgcacaaccactacacccagaagtcactgagcctgagcccagggaag

SEQ ID NO: 190 - protein, 450 aa, Artificial Sequence
  source: /note="Description of Artificial Sequence: Synthetic polypeptide"
QVQLVQSGAEVKKPGSSVKVSCKASGYTFSDYNMDWVRQAPGQGLEWMGQINPNNGGIFFNQKFQGRVTLTADKSTSTAYMELSSLRSEDTAVYYCAREAITTVGAMDYWGQGTLVTVSSASTKGPSVFPLAPSSKSTSGGTAALGCLVKDYFPEPVTVSWNSGALTSGVHTFPAVLQSSGLYSLSSVVTVPSSSLGTQTYICNVNHKPSNTKVDKRVEPKSCDKTHTCPPCPAPELLGGPSVFLFPPKPKDTLMISRTPEVTCVVVDVSHEDPEVKFNWYVDGVEVHNAKTKPREEQYNSTYRVVSVLTVLHQDWLNGKEYKCKVSNKALPAPIEKTISKAKGQPREPQVYTLPPSREEMTKNQVSLTCLVKGFYPSDIAVEWESNGQPENNYKTTPPVLDSDGSFFLYSKLTVDKSRWQQGNVFSCSVMHEALHNHYTQKSLSLSPGK

SEQ ID NO: 191 - DNA, 1347 bp, Artificial Sequence
  source: /note="Description of Artificial Sequence: Synthetic polynucleotide"
caggtgacactcaaagaatcaggacccggaatccttcagcccagccagaccttgtcgctgacttgttcgttctccggtttcagcctgaatacttatgggatgggtgtgtcatggatcaggcaaccgtccgggaaaggattggagtggctcgcgcacatctactgggacgatgacaaacgctacaatccttcgctgaagagccgattgacgatttccaaggatgcctcgaacaaccgggtatttcttaagatcacgtcggtcgatacggcagacacggcgacctattactgcgcccaaagagggtacgatgactattggggatattggggccaggggacactcgtcacaatttcagctgcctcaacaaaaggaccaagtgtgttcccactcgcccctagcagcaagagtacatccgggggcactgcagcactcggctgcctcgtcaaggattattttccagagccagtaaccgtgagctggaacagtggagcactcacttctggtgtccatacttttcctgctgtcctgcaaagctctggcctgtactcactcagctccgtcgtgaccgtgccatcttcatctctgggcactcagacctacatctgtaatgtaaaccacaagcctagcaatactaaggtcgataagcgggtggaacccaagagctgcgacaagactcacacttgtcccccatgccctgcccctgaacttctgggcggtcccagcgtctttttgttcccaccaaagcctaaagatactctgatgataagtagaacacccgaggtgacatgtgttgttgtagacgtttcccacgaggacccagaggttaagttcaactggtacgttgatggagtcgaagtacataatgctaagaccaagcctagagaggagcagtataatagtacataccgtgtagtcagtgttctcacagtgctgcaccaagactggctcaacggcaaagaatacaaatgcaaagtgtccaacaaagcactcccagcccctatcgagaagactattagtaaggcaaaggggcagcctcgtgaaccacaggtgtacactctgccacccagtagagaggaaatgacaaagaaccaagtctcattgacctgcctggtgaaaggcttctaccccagcgacatcgccgttgagtgggagagtaacggtcagcctgagaacaattacaagacaacccccccagtgctggatagtgacgggtctttctttctgtacagtaagctgactgtggacaagtcccgctggcagcagggtaacgtcttcagctgttccgtgatgcacgaggcattgcacaaccactacacccagaagtcactgagcctgagcccagggaag

SEQ ID NO: 192 - protein, 449 aa, Artificial Sequence
  source: /note="Description of Artificial Sequence: Synthetic polypeptide"
QVTLKESGPGILQPSQTLSLTCSFSGFSLNTYGMGVSWIRQPSGKGLEWLAHIYWDDDKRYNPSLKSRLTISKDASNNRVFLKITSVDTADTATYYCAQRGYDDYWGYWGQGTLVTISAASTKGPSVFPLAPSSKSTSGGTAALGCLVKDYFPEPVTVSWNSGALTSGVHTFPAVLQSSGLYSLSSVVTVPSSSLGTQTYICNVNHKPSNTKVDKRVEPKSCDKTHTCPPCPAPELLGGPSVFLFPPKPKDTLMISRTPEVTCVVVDVSHEDPEVKFNWYVDGVEVHNAKTKPREEQYNSTYRVVSVLTVLHQDWLNGKEYKCKVSNKALPAPIEKTISKAKGQPREPQVYTLPPSREEMTKNQVSLTCLVKGFYPSDIAVEWESNGQPENNYKTTPPVLDSDGSFFLYSKLTVDKSRWQQGNVFSCSVMHEALHNHYTQKSLSLSPGK

SEQ ID NO: 193 - DNA, 1347 bp, Artificial Sequence
  source: /note="Description of Artificial Sequence: Synthetic polynucleotide"
caggtgactttgaaagaatccggtcccgcattggtaaagccaacccagacacttacgctcacatgtacattttccggattcagcttgaacacttacgggatgggagtgtcgtggattcggcaacctccggggaaggctctggagtggctggcgcacatctactgggatgatgacaaaaggtataacccctcacttaaaacgagactgacgatctcgaaggacacaagcaagaatcaggtcgtcctcacgattacgaatgtagacccggtggatactgccgtctattactgcgcgcaacgcgggtatgatgactactggggatattggggtcagggcaccctcgtgaccatctcgtcagcctcaacaaaaggaccaagtgtgttcccactcgcccctagcagcaagagtacatccgggggcactgcagcactcggctgcctcgtcaaggattattttccagagccagtaaccgtgagctggaacagtggagcactcacttctggtgtccatacttttcctgctgtcctgcaaagctctggcctgtactcactcagctccgtcgtgaccgtgccatcttcatctctgggcactcagacctacatctgtaatgtaaaccacaagcctagcaatactaaggtcgataagcgggtggaacccaagagctgcgacaagactcacacttgtcccccatgccctgcccctgaacttctgggcggtcccagcgtctttttgttcccaccaaagcctaaagatactctgatgataagtagaacacccgaggtgacatgtgttgttgtagacgtttcccacgaggacccagaggttaagttcaactggtacgttgatggagtcgaagtacataatgctaagaccaagcctagagaggagcagtataatagtacataccgtgtagtcagtgttctcacagtgctgcaccaagactggctcaacggcaaagaatacaaatgcaaagtgtccaacaaagcactcccagcccctatcgagaagactattagtaaggcaaaggggcagcctcgtgaaccacaggtgtacactctgccacccagtagagaggaaatgacaaagaaccaagtctcattgacctgcctggtgaaaggcttctaccccagcgacatcgccgttgagtgggagagtaacggtcagcctgagaacaattacaagacaacccccccagtgctggatagtgacgggtctttctttctgtacagtaagctgactgtggacaagtcccgctggcagcagggtaacgtcttcagctgttccgtgatgcacgaggcattgcacaaccactacacccagaagtcactgagcctgagcccagggaag

SEQ ID NO: 194 - protein, 449 aa, Artificial Sequence
  source: /note="Description of Artificial Sequence: Synthetic polypeptide"
QVTLKESGPALVKPTQTLTLTCTFSGFSLNTYGMGVSWIRQPPGKALEWLAHIYWDDDKRYNPSLKTRLTISKDTSKNQVVLTITNVDPVDTAVYYCAQRGYDDYWGYWGQGTLVTISSASTKGPSVFPLAPSSKSTSGGTAALGCLVKDYFPEPVTVSWNSGALTSGVHTFPAVLQSSGLYSLSSVVTVPSSSLGTQTYICNVNHKPSNTKVDKRVEPKSCDKTHTCPPCPAPELLGGPSVFLFPPKPKDTLMISRTPEVTCVVVDVSHEDPEVKFNWYVDGVEVHNAKTKPREEQYNSTYRVVSVLTVLHQDWLNGKEYKCKVSNKALPAPIEKTISKAKGQPREPQVYTLPPSREEMTKNQVSLTCLVKGFYPSDIAVEWESNGQPENNYKTTPPVLDSDGSFFLYSKLTVDKSRWQQGNVFSCSVMHEALHNHYTQKSLSLSPGK

SEQ ID NO: 195 - DNA, 1347 bp, Artificial Sequence
  source: /note="Description of Artificial Sequence: Synthetic polynucleotide"
caagtaacgctcaaggagtccggacccaccttggtgaagccgacgcagaccttgactcttacgtgcactttctcggggttttcactgaatacgtacgggatgggtgtctcatggatcaggcaacctccggggaaaggattggaatggctggcgcacatctactgggatgacgataagagatataacccaagcctcaagtcgcggctcaccattacaaaagatacatcgaaaaatcaggtcgtacttactatcacgaacatggaccccgtggacacagcaacatattactgtgcccagcgcggctatgacgattattggggttactggggacagggaacactggtcacggtgtccagcgcctcaacaaaaggaccaagtgtgttcccactcgcccctagcagcaagagtacatccgggggcactgcagcactcggctgcctcgtcaaggattattttccagagccagtaaccgtgagctggaacagtggagcactcacttctggtgtccatacttttcctgctgtcctgcaaagctctggcctgtactcactcagctccgtcgtgaccgtgccatcttcatctctgggcactcagacctacatctgtaatgtaaaccacaagcctagcaatactaaggtcgataagcgggtggaacccaagagctgcgacaagactcacacttgtcccccatgccctgcccctgaacttctgggcggtcccagcgtctttttgttcccaccaaagcctaaagatactctgatgataagtagaacacccgaggtgacatgtgttgttgtagacgtttcccacgaggacccagaggttaagttcaactggtacgttgatggagtcgaagtacataatgctaagaccaagcctagagaggagcagtataatagtacataccgtgtagtcagtgttctcacagtgctgcaccaagactggctcaacggcaaagaatacaaatgcaaagtgtccaacaaagcactcccagcccctatcgagaagactattagtaaggcaaaggggcagcctcgtgaaccacaggtgtacactctgccacccagtagagaggaaatgacaaagaaccaagtctcattgacctgcctggtgaaaggcttctaccccagcgacatcgccgttgagtgggagagtaacggtcagcctgagaacaattacaagacaacccccccagtgctggatagtgacgggtctttctttctgtacagtaagctgactgtggacaagtcccgctggcagcagggtaacgtcttcagctgttccgtgatgcacgaggcattgcacaaccactacacccagaagtcactgagcctgagcccagggaag

SEQ ID NO: 196 - protein, 449 aa, Artificial Sequence
  source: /note="Description of Artificial Sequence: Synthetic polypeptide"
QVTLKESGPTLVKPTQTLTLTCTFSGFSLNTYGMGVSWIRQPPGKGLEWLAHIYWDDDKRYNPSLKSRLTITKDTSKNQVVLTITNMDPVDTATYYCAQRGYDDYWGYWGQGTLVTVSSASTKGPSVFPLAPSSKSTSGGTAALGCLVKDYFPEPVTVSWNSGALTSGVHTFPAVLQSSGLYSLSSVVTVPSSSLGTQTYICNVNHKPSNTKVDKRVEPKSCDKTHTCPPCPAPELLGGPSVFLFPPKPKDTLMISRTPEVTCVVVDVSHEDPEVKFNWYVDGVEVHNAKTKPREEQYNSTYRVVSVLTVLHQDWLNGKEYKCKVSNKALPAPIEKTISKAKGQPREPQVYTLPPSREEMTKNQVSLTCLVKGFYPSDIAVEWESNGQPENNYKTTPPVLDSDGSFFLYSKLTVDKSRWQQGNVFSCSVMHEALHNHYTQKSLSLSPGK

SEQ ID NO: 197 - DNA, 1347 bp, Artificial Sequence
  source: /note="Description of Artificial Sequence: Synthetic polynucleotide"
caggtcacgctgaaagagtcaggtcccggaatccttcaaccttcgcagacattgtcactcacatgttccttctccgggttctcgctctcgacttatggcatgggtgtaggatggattcggcagcccagcgggaaggggcttgagtggttggcggatatctggtgggacgacgacaaatactacaatccgagcctgaagtcccgcctcaccatttcgaaagatacgtcatcaaacgaagtctttttgaagatcgccatcgtggacacggcggatacagcgacgtattactgcgccagaaggggacactacagcgcaatggattattggggacaggggacctcggtgactgtgtcgtccgcctcaacaaaaggaccaagtgtgttcccactcgcccctagcagcaagagtacatccgggggcactgcagcactcggctgcctcgtcaaggattattttccagagccagtaaccgtgagctggaacagtggagcactcacttctggtgtccatacttttcctgctgtcctgcaaagctctggcctgtactcactcagctccgtcgtgaccgtgccatcttcatctctgggcactcagacctacatctgtaatgtaaaccacaagcctagcaatactaaggtcgataagcgggtggaacccaagagctgcgacaagactcacacttgtcccccatgccctgcccctgaacttctgggcggtcccagcgtctttttgttcccaccaaagcctaaagatactctgatgataagtagaacacccgaggtgacatgtgttgttgtagacgtttcccacgaggacccagaggttaagttcaactggtacgttgatggagtcgaagtacataatgctaagaccaagcctagagaggagcagtataatagtacataccgtgtagtcagtgttctcacagtgctgcaccaagactggctcaacggcaaagaatacaaatgcaaagtgtccaacaaagcactcccagcccctatcgagaagactattagtaaggcaaaggggcagcctcgtgaaccacaggtgtacactctgccacccagtagagaggaaatgacaaagaaccaagtctcattgacctgcctggtgaaaggcttctaccccagcgacatcgccgttgagtgggagagtaacggtcagcctgagaacaattacaagacaacccccccagtgctggatagtgacgggtctttctttctgtacagtaagctgactgtggacaagtcccgctggcagcagggtaacgtcttcagctgttccgtgatgcacgaggcattgcacaaccactacacccagaagtcactgagcctgagcccagggaag

SEQ ID NO: 198 - protein, 449 aa, Artificial Sequence
  source: /note="Description of Artificial Sequence: Synthetic polypeptide"
QVTLKESGPGILQPSQTLSLTCSFSGFSLSTYGMGVGWIRQPSGKGLEWLADIWWDDDKYYNPSLKSRLTISKDTSSNEVFLKIAIVDTADTATYYCARRGHYSAMDYWGQGTSVTVSSASTKGPSVFPLAPSSKSTSGGTAALGCLVKDYFPEPVTVSWNSGALTSGVHTFPAVLQSSGLYSLSSVVTVPSSSLGTQTYICNVNHKPSNTKVDKRVEPKSCDKTHTCPPCPAPELLGGPSVFLFPPKPKDTLMISRTPEVTCVVVDVSHEDPEVKFNWYVDGVEVHNAKTKPREEQYNSTYRVVSVLTVLHQDWLNGKEYKCKVSNKALPAPIEKTISKAKGQPREPQVYTLPPSREEMTKNQVSLTCLVKGFYPSDIAVEWESNGQPENNYKTTPPVLDSDGSFFLYSKLTVDKSRWQQGNVFSCSVMHEALHNHYTQKSLSLSPGK

SEQ ID NO: 199 - DNA, 1347 bp, Artificial Sequence
  source: /note="Description of Artificial Sequence: Synthetic polynucleotide"
cagatcactttgaaagaaagcggaccgaccttggtcaagcccacacaaaccctcacgctcacgtgtacattttcggggttctcgctttcaacttacgggatgggagtagggtggattcgccagccgcctggtaaagcgttggagtggcttgcagacatctggtgggacgacgataagtactataatccctcgctcaagtccagactgaccatcacgaaagatacgagcaagaaccaggtcgtgctgacaatgactaacatggacccagtggatacggctacatattactgcgccaggcggggtcactactcagcgatggattattggggccagggaacactggtaacggtgtcgtccgcctcaacaaaaggaccaagtgtgttcccactcgcccctagcagcaagagtacatccgggggcactgcagcactcggctgcctcgtcaaggattattttccagagccagtaaccgtgagctggaacagtggagcactcacttctggtgtccatacttttcctgctgtcctgcaaagctctggcctgtactcactcagctccgtcgtgaccgtgccatcttcatctctgggcactcagacctacatctgtaatgtaaaccacaagcctagcaatactaaggtcgataagcgggtggaacccaagagctgcgacaagactcacacttgtcccccatgccctgcccctgaacttctgggcggtcccagcgtctttttgttcccaccaaagcctaaagatactctgatgataagtagaacacccgaggtgacatgtgttgttgtagacgtttcccacgaggacccagaggttaagttcaactggtacgttgatggagtcgaagtacataatgctaagaccaagcctagagaggagcagtataatagtacataccgtgtagtcagtgttctcacagtgctgcaccaagactggctcaacggcaaagaatacaaatgcaaagtgtccaacaaagcactcccagcccctatcgagaagactattagtaaggcaaaggggcagcctcgtgaaccacaggtgtacactctgccacccagtagagaggaaatgacaaagaaccaagtctcattgacctgcctggtgaaaggcttctaccccagcgacatcgccgttgagtgggagagtaacggtcagcctgagaacaattacaagacaacccccccagtgctggatagtgacgggtctttctttctgtacagtaagctgactgtggacaagtcccgctggcagcagggtaacgtcttcagctgttccgtgatgcacgaggcattgcacaaccactacacccagaagtcactgagcctgagcccagggaag

SEQ ID NO: 200 - protein, 449 aa, Artificial Sequence
  source: /note="Description of Artificial Sequence: Synthetic polypeptide"
QITLKESGPTLVKPTQTLTLTCTFSGFSLSTYGMGVGWIRQPPGKALEWLADIWWDDDKYYNPSLKSRLTITKDTSKNQVVLTMTNMDPVDTATYYCARRGHYSAMDYWGQGTLVTVSSASTKGPSVFPLAPSSKSTSGGTAALGCLVKDYFPEPVTVSWNSGALTSGVHTFPAVLQSSGLYSLSSVVTVPSSSLGTQTYICNVNHKPSNTKVDKRVEPKSCDKTHTCPPCPAPELLGGPSVFLFPPKPKDTLMISRTPEVTCVVVDVSHEDPEVKFNWYVDGVEVHNAKTKPREEQYNSTYRVVSVLTVLHQDWLNGKEYKCKVSNKALPAPIEKTISKAKGQPREPQVYTLPPSREEMTKNQVSLTCLVKGFYPSDIAVEWESNGQPENNYKTTPPVLDSDGSFFLYSKLTVDKSRWQQGNVFSCSVMHEALHNHYTQKSLSLSPGK

SEQ ID NO: 201 - DNA, 1347 bp, Artificial Sequence
  source: /note="Description of Artificial Sequence: Synthetic polynucleotide"
caagtgactctcaaggagtccggacccgccctggtcaaaccaacgcagacactgacgctcacatgcaccttcagcggattttcgttgtcaacgtacggcatgggtgtggggtggattcgccagcctccggggaaagcccttgaatggttggcggacatctggtgggatgatgacaagtactataatccctcacttaagtcacggttgacgatctcgaaagacaccagcaagaaccaggtagtgctgacaatgactaacatggacccggtcgatacagcggtctactattgtgctagaaggggacactactccgcaatggattattggggtcaggggacgctcgtaaccgtgtcgtcggcctcaacaaaaggaccaagtgtgttcccactcgcccctagcagcaagagtacatccgggggcactgcagcactcggctgcctcgtcaaggattattttccagagccagtaaccgtgagctggaacagtggagcactcacttctggtgtccatacttttcctgctgtcctgcaaagctctggcctgtactcactcagctccgtcgtgaccgtgccatcttcatctctgggcactcagacctacatctgtaatgtaaaccacaagcctagcaatactaaggtcgataagcgggtggaacccaagagctgcgacaagactcacacttgtcccccatgccctgcccctgaacttctgggcggtcccagcgtctttttgttcccaccaaagcctaaagatactctgatgataagtagaacacccgaggtgacatgtgttgttgtagacgtttcccacgaggacccagaggttaagttcaactggtacgttgatggagtcgaagtacataatgctaagaccaagcctagagaggagcagtataatagtacataccgtgtagtcagtgttctcacagtgctgcaccaagactggctcaacggcaaagaatacaaatgcaaagtgtccaacaaagcactcccagcccctatcgagaagactattagtaaggcaaaggggcagcctcgtgaaccacaggtgtacactctgccacccagtagagaggaaatgacaaagaaccaagtctcattgacctgcctggtgaaaggcttctaccccagcgacatcgccgttgagtgggagagtaacggtcagcctgagaacaattacaagacaacccccccagtgctggatagtgacgggtctttctttctgtacagtaagctgactgtggacaagtcccgctggcagcagggtaacgtcttcagctgttccgtgatgcacgaggcattgcacaaccactacacccagaagtcactgagcctgagcccagggaag

SEQ ID NO: 202 - protein, 449 aa, Artificial Sequence
  source: /note="Description of Artificial Sequence: Synthetic polypeptide"
QVTLKESGPALVKPTQTLTLTCTFSGFSLSTYGMGVGWIRQPPGKALEWLADIWWDDDKYYNPSLKSRLTISKDTSKNQVVLTMTNMDPVDTAVYYCARRGHYSAMDYWGQGTLVTVSSASTKGPSVFPLAPSSKSTSGGTAALGCLVKDYFPEPVTVSWNSGALTSGVHTFPAVLQSSGLYSLSSVVTVPSSSLGTQTYICNVNHKPSNTKVDKRVEPKSCDKTHTCPPCPAPELLGGPSVFLFPPKPKDTLMISRTPEVTCVVVDVSHEDPEVKFNWYVDGVEVHNAKTKPREEQYNSTYRVVSVLTVLHQDWLNGKEYKCKVSNKALPAPIEKTISKAKGQPREPQVYTLPPSREEMTKNQVSLTCLVKGFYPSDIAVEWESNGQPENNYKTTPPVLDSDGSFFLYSKLTVDKSRWQQGNVFSCSVMHEALHNHYTQKSLSLSPGK

SEQ ID NO: 203 - DNA, 642 bp, Artificial Sequence
  source: /note="Description of Artificial Sequence: Synthetic polynucleotide"
gacatccaaatgacccagtcacccgcgagcctttcggcgtcggtcggagaaacggtcacgatcacgtgccggacatcagagaatctccataactacctcgcgtggtatcaacagaagcaggggaagtcgccccagttgcttgtatacgatgcgaaaacgttggcggatggggtgccgtccagattctcgggatcgggctcggggacgcagtactcgctcaagatcaattcgctgcagccggaggactttgggtcgtactattgtcagcatttttggtcatcaccgtatacatttggaggtggaacgaaacttgagattaagcgcacagttgctgcccccagcgtgttcattttcccacctagcgatgagcagctgaaaagcggtactgcctctgtcgtatgcttgctcaacaacttttacccacgtgaggctaaggtgcagtggaaagtggataatgcacttcaatctggaaacagtcaagagtccgtgacagaacaggacagcaaagactcaacttattcactctcttccaccctgactctgtccaaggcagactatgaaaaacacaaggtatacgcctgcgaggttacacaccagggtttgtctagtcctgtcaccaagtccttcaataggggcgaatgt

SEQ ID NO: 204 - protein, 214 aa, Artificial Sequence
  source: /note="Description of Artificial Sequence: Synthetic polypeptide"
DIQMTQSPASLSASVGETVTITCRTSENLHNYLAWYQQKQGKSPQLLVYDAKTLADGVPSRFSGSGSGTQYSLKINSLQPEDFGSYYCQHFWSSPYTFGGGTKLEIKRTVAAPSVFIFPPSDEQLKSGTASVVCLLNNFYPREAKVQWKVDNALQSGNSQESVTEQDSKDSTYSLSSTLTLSKADYEKHKVYACEVTHQGLSSPVTKSFNRGEC

SEQ ID NO: 205 - DNA, 642 bp, Artificial Sequence
  source: /note="Description of Artificial Sequence: Synthetic polynucleotide"
gacatccaaatgacccagtcgccgtcgtcgctttcagcgtcggtaggggatcgggtcacaattacgtgccgaacgtcagagaatttgcataactacctcgcgtggtatcagcagaagcccgggaagtcaccgaaactccttgtctacgatgcgaaaacgctggcggatggagtgccgtcgagattctcgggaagcggatccggtacggactatacgcttacgatctcatcgctccagcccgaggactttgcgacgtactattgtcagcatttttggtcgtcgccctacacatttgggcaggggaccaagttggaaatcaagcgcacagttgctgcccccagcgtgttcattttcccacctagcgatgagcagctgaaaagcggtactgcctctgtcgtatgcttgctcaacaacttttacccacgtgaggctaaggtgcagtggaaagtggataatgcacttcaatctggaaacagtcaagagtccgtgacagaacaggacagcaaagactcaacttattcactctcttccaccctgactctgtccaaggcagactatgaaaaacacaaggtatacgcctgcgaggttacacaccagggtttgtctagtcctgtcaccaagtccttcaataggggcgaatgt

SEQ ID NO: 206 - protein, 214 aa, Artificial Sequence
  source: /note="Description of Artificial Sequence: Synthetic polypeptide"
DIQMTQSPSSLSASVGDRVTITCRTSENLHNYLAWYQQKPGKSPKLLVYDAKTLADGVPSRFSGSGSGTDYTLTISSLQPEDFATYYCQHFWSSPYTFGQGTKLEIKRTVAAPSVFIFPPSDEQLKSGTASVVCLLNNFYPREAKVQWKVDNALQSGNSQESVTEQDSKDSTYSLSSTLTLSKADYEKHKVYACEVTHQGLSSPVTKSFNRGEC

SEQ ID NO: 207 - DNA, 642 bp, Artificial Sequence
  source: /note="Description of Artificial Sequence: Synthetic polynucleotide"
gacatccaaatgacccagtcgccgtcgtcgctttcagcgtcggtaggggatcgggtcacaattacgtgccgaacgtcagagaatttgcataactacctcgcgtggtatcagcagaagcccgggaaggccccgaaactccttatctacgatgcgaaaacgctggcggatggagtgccgtcgagattctcgggaagcggatccggtacggactatacgcttacgatctcatcgctccagcccgaggactttgcgacgtactattgtcagcatttttggtcgtcgccctacacatttgggcaggggaccaagttggaaatcaagcgcacagttgctgcccccagcgtgttcattttcccacctagcgatgagcagctgaaaagcggtactgcctctgtcgtatgcttgctcaacaacttttacccacgtgaggctaaggtgcagtggaaagtggataatgcacttcaatctggaaacagtcaagagtccgtgacagaacaggacagcaaagactcaacttattcactctcttccaccctgactctgtccaaggcagactatgaaaaacacaaggtatacgcctgcgaggttacacaccagggtttgtctagtcctgtcaccaagtccttcaataggggcgaatgt

SEQ ID NO: 208 - protein, 214 aa, Artificial Sequence
  source: /note="Description of Artificial Sequence: Synthetic polypeptide"
DIQMTQSPSSLSASVGDRVTITCRTSENLHNYLAWYQQKPGKAPKLLIYDAKTLADGVPSRFSGSGSGTDYTLTISSLQPEDFATYYCQHFWSSPYTFGQGTKLEIKRTVAAPSVFIFPPSDEQLKSGTASVVCLLNNFYPREAKVQWKVDNALQSGNSQESVTEQDSKDSTYSLSSTLTLSKADYEKHKVYACEVTHQGLSSPVTKSFNRGEC

SEQ ID NO: 209 - DNA, 642 bp, Artificial Sequence
  source: /note="Description of Artificial Sequence: Synthetic polynucleotide"
gacatccaaatgacccagtcgccgtcgtcgctttcagcgtcggtaggggatcgggtcacaattacgtgccgaacgtcagagaatttgcataactacctcgcgtggtatcagcagaagcccgggaagtcaccgaaactccttatctacgatgcgaaaacgctggcggatggagtgccgtcgagattctcgggaagcggatccggtacggactatacgcttacgatctcatcgctccagcccgaggactttgcgacgtactattgtcagcatttttggtcgtcgccctacacatttgggcaggggaccaagttggaaatcaagcgcacagttgctgcccccagcgtgttcattttcccacctagcgatgagcagctgaaaagcggtactgcctctgtcgtatgcttgctcaacaacttttacccacgtgaggctaaggtgcagtggaaagtggataatgcacttcaatctggaaacagtcaagagtccgtgacagaacaggacagcaaagactcaacttattcactctcttccaccctgactctgtccaaggcagactatgaaaaacacaaggtatacgcctgcgaggttacacaccagggtttgtctagtcctgtcaccaagtccttcaataggggcgaatgt

SEQ ID NO: 210 - protein, 214 aa, Artificial Sequence
  source: /note="Description of Artificial Sequence: Synthetic polypeptide"
DIQMTQSPSSLSASVGDRVTITCRTSENLHNYLAWYQQKPGKSPKLLIYDAKTLADGVPSRFSGSGSGTDYTLTISSLQPEDFATYYCQHFWSSPYTFGQGTKLEIKRTVAAPSVFIFPPSDEQLKSGTASVVCLLNNFYPREAKVQWKVDNALQSGNSQESVTEQDSKDSTYSLSSTLTLSKADYEKHKVYACEVTHQGLSSPVTKSFNRGEC

SEQ ID NO: 211 - DNA, 642 bp, Artificial Sequence
  source: /note="Description of Artificial Sequence: Synthetic polynucleotide"
gatatcgtcatgacccagtcccagaagttcatgtcaacttcagtgggagacagagtgtccgtcacatgtaaagcctcgcaaaatgtgggaaccaacgtagcgtggttccagcagaaacctggccaatcaccgaaggcactgatctactcggccagctataggtactcgggagtaccagatcggtttacggggtcggggagcgggacggactttatcctcactatttccaatgtccagtcggaggaccttgcggaatacttctgccagcagtataacaactatcccctcacgtttggtgctggtacaaaattggagttgaagcgcacagttgctgcccccagcgtgttcattttcccacctagcgatgagcagctgaaaagcggtactgcctctgtcgtatgcttgctcaacaacttttacccacgtgaggctaaggtgcagtggaaagtggataatgcacttcaatctggaaacagtcaagagtccgtgacagaacaggacagcaaagactcaacttattcactctcttccaccctgactctgtccaaggcagactatgaaaaacacaaggtatacgcctgcgaggttacacaccagggtttgtctagtcctgtcaccaagtccttcaataggggcgaatgt

SEQ ID NO: 212 - protein, 214 aa, Artificial Sequence
  source: /note="Description of Artificial Sequence: Synthetic polypeptide"
DIVMTQSQKFMSTSVGDRVSVTCKASQNVGTNVAWFQQKPGQSPKALIYSASYRYSGVPDRFTGSGSGTDFILTISNVQSEDLAEYFCQQYNNYPLTFGAGTKLELKRTVAAPSVFIFPPSDEQLKSGTASVVCLLNNFYPREAKVQWKVDNALQSGNSQESVTEQDSKDSTYSLSSTLTLSKADYEKHKVYACEVTHQGLSSPVTKSFNRGEC

SEQ ID NO: 213 - DNA, 642 bp, Artificial Sequence
  source: /note="Description of Artificial Sequence: Synthetic polynucleotide"
gacatccaaatgacccaatcgccctcctccctctccgcatcagtaggggaccgcgtcacaattacttgcaaagcgtcgcagaacgtcggaacgaatgtggcgtggtttcagcagaagcccggaaaagctccgaagagcttgatctactcggcctcatataggtattcgggtgtgccgagccggtttagcgggtcggggtcaggtactgatttcacgctcacaatttcatcgttgcagccagaagatttcgccacatattactgtcagcagtacaacaattaccctctgacgttcggccagggaaccaaacttgagatcaagcgcacagttgctgcccccagcgtgttcattttcccacctagcgatgagcagctgaaaagcggtactgcctctgtcgtatgcttgctcaacaacttttacccacgtgaggctaaggtgcagtggaaagtggataatgcacttcaatctggaaacagtcaagagtccgtgacagaacaggacagcaaagactcaacttattcactctcttccaccctgactctgtccaaggcagactatgaaaaacacaaggtatacgcctgcgaggttacacaccagggtttgtctagtcctgtcaccaagtccttcaataggggcgaatgt

SEQ ID NO: 214 - protein, 214 aa, Artificial Sequence
  source: /note="Description of Artificial Sequence: Synthetic polypeptide"
DIQMTQSPSSLSASVGDRVTITCKASQNVGTNVAWFQQKPGKAPKSLIYSASYRYSGVPSRFSGSGSGTDFTLTISSLQPEDFATYYCQQYNNYPLTFGQGTKLEIKRTVAAPSVFIFPPSDEQLKSGTASVVCLLNNFYPREAKVQWKVDNALQSGNSQESVTEQDSKDSTYSLSSTLTLSKADYEKHKVYACEVTHQGLSSPVTKSFNRGEC

SEQ ID NO: 215 - DNA, 642 bp, Artificial Sequence
  source: /note="Description of Artificial Sequence: Synthetic polynucleotide"
gacatcgtgatgacacagtcacagaaattcatgtccacatccgtcggtgatagagtatccgtcacgtgtaaggcctcgcaaaacgtaggaactaatgtggcgtggtatcaacagaagccaggacagtcacccaaagcactcatctacagcccctcatatcggtacagcggggtgccggacaggttcacgggatcggggagcgggaccgattttacactgaccatttcgaatgtccagtcggaggaccttgcggaatacttctgccagcagtataactcgtaccctcacacgtttggaggtggcactaagttggagatgaaacgcacagttgctgcccccagcgtgttcattttcccacctagcgatgagcagctgaaaagcggtactgcctctgtcgtatgcttgctcaacaacttttacccacgtgaggctaaggtgcagtggaaagtggataatgcacttcaatctggaaacagtcaagagtccgtgacagaacaggacagcaaagactcaacttattcactctcttccaccctgactctgtccaaggcagactatgaaaaacacaaggtatacgcctgcgaggttacacaccagggtttgtctagtcctgtcaccaagtccttcaataggggcgaatgt

SEQ ID NO: 216 - protein, 214 aa, Artificial Sequence
  source: /note="Description of Artificial Sequence: Synthetic polypeptide"
DIVMTQSQKFMSTSVGDRVSVTCKASQNVGTNVAWYQQKPGQSPKALIYSPSYRYSGVPDRFTGSGSGTDFTLTISNVQSEDLAEYFCQQYNSYPHTFGGGTKLEMKRTVAAPSVFIFPPSDEQLKSGTASVVCLLNNFYPREAKVQWKVDNALQSGNSQESVTEQDSKDSTYSLSSTLTLSKADYEKHKVYACEVTHQGLSSPVTKSFNRGEC

SEQ ID NO: 217 - DNA, 642 bp, Artificial Sequence
  source: /note="Description of Artificial Sequence: Synthetic polynucleotide"
gatatccagatgacacagtcaccctcgtcgctctcagcttccgtaggcgacagggtcactattacgtgtaaagcatcacagaacgtcggaacgaatgtggcgtggtttcagcagaagcccgggaagagccccaaagcgcttatctactccccgtcgtatcggtattccggtgtgccaagcagattttcggggtcaggttcgggaactgactttaccctgaccatctcgtccctccaaccggaagatttcgccacgtacttctgccagcagtacaacagctatcctcacacattcggacaagggacaaagttggagattaaacgcacagttgctgcccccagcgtgttcattttcccacctagcgatgagcagctgaaaagcggtactgcctctgtcgtatgcttgctcaacaacttttacccacgtgaggctaaggtgcagtggaaagtggataatgcacttcaatctggaaacagtcaagagtccgtgacagaacaggacagcaaagactcaacttattcactctcttccaccctgactctgtccaaggcagactatgaaaaacacaaggtatacgcctgcgaggttacacaccagggtttgtctagtcctgtcaccaagtccttcaataggggcgaatgt

SEQ ID NO: 218 - protein, 214 aa, Artificial Sequence
  source: /note="Description of Artificial Sequence: Synthetic polypeptide"
DIQMTQSPSSLSASVGDRVTITCKASQNVGTNVAWFQQKPGKSPKALIYSPSYRYSGVPSRFSGSGSGTDFTLTISSLQPEDFATYFCQQYNSYPHTFGQGTKLEIKRTVAAPSVFIFPPSDEQLKSGTASVVCLLNNFYPREAKVQWKVDNALQSGNSQESVTEQDSKDSTYSLSSTLTLSKADYEKHKVYACEVTHQGLSSPVTKSFNRGEC

SEQ ID NO: 219 - DNA, 1035 bp, Artificial Sequence
  source: /note="Description of Artificial Sequence: Synthetic polynucleotide"
gggtgtaaaccctgcatctgcacggtgccggaggtgtcctccgtctttatcttccctcccaaacccaaggatgtgctgacaatcactttgactccaaaagtcacatgcgtagtcgtggacatctcgaaagacgacccggaagtgcagttctcgtggtttgttgatgatgtagaagtgcataccgctcaaacccagccgagggaagaacagtttaacagcacgtttaggagtgtgtcggaactgcccattatgcaccaggattggcttaatgggaaggagttcaaatgtcgcgtgaatagtgcggcgttcccagcccctattgaaaagactatttccaaaacgaagggtcggcccaaagctccccaagtatacacaatccctccgccgaaagaacaaatggcaaaagacaaagtgagtttgacgtgcatgatcacggactttttcccggaggatatcaccgtcgaatggcaatggaatgggcaacctgccgaaaactacaagaatacacaacccattatggataccgatggatcgtatttcgtctactcaaagttgaacgtacagaagtcaaattgggaggcagggaatacgttcacttgcagtgttttgcacgaaggcctccataaccaccatacggaaaagtcactgtcgcactccccgggaaaaatcgagggcagaatggatggtggaggagggtcggcgcgcaacggggaccactgtccgctcgggcccgggcgttgctgccgtctgcacacggtccgcgcgtcgctggaagacctgggctgggccgattgggtgctgtcgccacgggaggtgcaagtgaccatgtgcatcggcgcgtgcccgagccagttccgggcggcaaacatgcacgcgcagatcaagacgagcctgcaccgcctgaagcccgacacggtgccagcgccctgctgcgtgcccgccagctacaatcccatggtgctcattcaaaagaccgacaccggggtgtcgctccagacctatgatgacttgttagccaaagactgccactgcata

SEQ ID NO: 220 - protein, 345 aa, Artificial Sequence
  source: /note="Description of Artificial Sequence: Synthetic polypeptide"
GCKPCICTVPEVSSVFIFPPKPKDVLTITLTPKVTCVVVDISKDDPEVQFSWFVDDVEVHTAQTQPREEQFNSTFRSVSELPIMHQDWLNGKEFKCRVNSAAFPAPIEKTISKTKGRPKAPQVYTIPPPKEQMAKDKVSLTCMITDFFPEDITVEWQWNGQPAENYKNTQPIMDTDGSYFVYSKLNVQKSNWEAGNTFTCSVLHEGLHNHHTEKSLSHSPGKIEGRMDGGGGSARNGDHCPLGPGRCCRLHTVRASLEDLGWADWVLSPREVQVTMCIGACPSQFRAANMHAQIKTSLHRLKPDTVPAPCCVPASYNPMVLIQKTDTGVSLQTYDDLLAKDCHCI

SEQ ID NO: 221 - DNA, 1026 bp, Artificial Sequence
  source: /note="Description of Artificial Sequence: Synthetic polynucleotide"
tcgaaacccacttgccctcctccggagctgttgggcggaccctccgtgtttatctttcccccgaagccgaaagatacccttatgatctcacggacgccggaggtcacttgcgtagtagtggatgtgtcggaggatgaccccgaagtccagttcacctggtatatcaataacgagcaagtgaggacagcgaggcccccacttagggagcagcagttcaactccacaattcgggtcgtcagcactttgcccatcgctcatgaggactggctccgcggaaaagagttcaagtgtaaggtgcataacaaggcattgccagcgcctattgaaaagacaatctcgaaggcgcgagggcagccgctcgagcccaaagtgtatacgatgggacccccgagggaagaattgtcgtcgcgctcagtaagccttacgtgcatgattaacggtttctaccctagcgacatcagcgtagagtgggaaaagaatggaaaggcggaggataactacaagacgactcccgcggtgctggattcggatgggtcgtactttctgtatagcaaattgtcagtcccgacctcagaatggcagaggggtgacgtgttcacgtgctccgtgatgcacgaagcacttcacaatcactacacccagaaatcaatctcgcggtccccaggcaaaggtggaggagggtcggctcacgcccaccctcgcgattcgtgtccgctggggcctggtagatgctgtcatctcgagacagtccaggccacgctggaggacctcgggtggtcagactgggtcctgtccccacgacaactgcagctttcgatgtgcgtgggggaatgtccgcacttgtacagatcggcgaatacccacgctcagattaaggcacgactccatggtttgcagccagataaagtccccgcaccttgctgtgtccccagctcatatactcctgtcgtactcatgcatcggacagacagcggcgtgtcgcttcaaacgtatgacgacctcgtagcgagaggatgtcattgcgcc

SEQ ID NO: 222 - protein, 342 aa, Artificial Sequence
  source: /note="Description of Artificial Sequence: Synthetic polypeptide"
SKPTCPPPELLGGPSVFIFPPKPKDTLMISRTPEVTCVVVDVSEDDPEVQFTWYINNEQVRTARPPLREQQFNSTIRVVSTLPIAHEDWLRGKEFKCKVHNKALPAPIEKTISKARGQPLEPKVYTMGPPREELSSRSVSLTCMINGFYPSDISVEWEKNGKAEDNYKTTPAVLDSDGSYFLYSKLSVPTSEWQRGDVFTCSVMHEALHNHYTQKSISRSPGKGGGGSAHAHPRDSCPLGPGRCCHLETVQATLEDLGWSDWVLSPRQLQLSMCVGECPHLYRSANTHAQIKARLHGLQPDKVPAPCCVPSSYTPVVLMHRTDSGVSLQTYDDLVARGCHCA

SEQ ID NO: 223 - protein, 350 aa, Artificial Sequence
  source: /note="Description of Artificial Sequence: Synthetic polypeptide"
DKTHTCPPCPAPELLGGPSVFLFPPKPKDTLMISRTPEVTCVVVDVSHEDPEVKFNWYVDGVEVHNAKTKPREEQYNSTYRVVSVLTVLHQDWLNGKEYKCKVSNKALPAPIEKTISKAKGQPREPQVYTLPPSREEMTKNQVSLTCLVKGFYPSDIAVEWESNGQPENNYKTTPPVLDSDGSFFLYSKLTVDKSRWQQGNVFSCSVMHEALHNHYTQKSLSLSPGKIEGRMDGGGGSARNGDHCPLGPGRCCRLHTVRASLEDLGWADWVLSPREVQVTMCIGACPSQFRAANMHAQIKTSLHRLKPDTVPAPCCVPASYNPMVLIQKTDTGVSLQTYDDLLAKDCHCI

SEQ ID NO: 224 - protein, 344 aa, Artificial Sequence
  source: /note="Description of Artificial Sequence: Synthetic polypeptide"
DKTHTCPPCPAPELLGGPSVFLFPPKPKDTLMISRTPEVTCVVVDVSHEDPEVKFNWYVDGVEVHNAKTKPREEQYNSTYRVVSVLTVLHQDWLNGKEYKCKVSNKALPAPIEKTISKAKGQPREPQVYTLPPSREEMTKNQVSLTCLVKGFYPSDIAVEWESNGQPENNYKTTPPVLDSDGSFFLYSKLTVDKSRWQQGNVFSCSVMHEALHNHYTQKSLSLSPGKGGGGSARNGDHCPLGPGRCCRLHTVRASLEDLGWADWVLSPREVQVTMCIGACPSQFRAANMHAQIKTSLHRLKPDTVPAPCCVPASYNPMVLIQKTDTGVSLQTYDDLLAKDCHCI

SEQ ID NO: 225 - DNA, 22 bp, Artificial Sequence
  source: /note="Description of Artificial Sequence: Synthetic primer"
ctaatacgactcactatagggc

SEQ ID NO: 226 - DNA, 21 bp, Artificial Sequence
  source: /note="Description of Artificial Sequence: Synthetic primer"
tatgcaaggcttacaaccaca

SEQ ID NO: 227 - DNA, 21 bp, Artificial Sequence
  source: /note="Description of Artificial Sequence: Synthetic primer"
aggacaggggttgattgttga

SEQ ID NO: 228 - DNA, 27 bp, Artificial Sequence
  source: /note="Description of Artificial Sequence: Synthetic primer"
ctcattcctgttgaagctcttgacaat

SEQ ID NO: 229 - DNA, 23 bp, Artificial Sequence
  source: /note="Description of Artificial Sequence: Synthetic primer"
aagcagtggtatcaacgcagagt

SEQ ID NO: 230 - DNA, 23 bp, Artificial Sequence
  source: /note="Description of Artificial Sequence: Synthetic primer"
cgactgaggcacctccagatgtt

SEQ ID NO: 231 - DNA, 17 bp, Artificial Sequence
  source: /note="Description of Artificial Sequence: Synthetic primer"
gtaaaacgacggccagt

SEQ ID NO: 232 - DNA, 18 bp, Artificial Sequence
  source: /note="Description of Artificial Sequence: Synthetic primer"
caggaaacagctatgacc

SEQ ID NO: 233 - DNA, 45 bp, Artificial Sequence
  source: /note="Description of Artificial Sequence: Synthetic primer"
ctaatacgactcactatagggcaagcagtggtatcaacgcagagt

SEQ ID NO: 234 - protein, 7 aa, Artificial Sequence
  source: /note="Description of Artificial Sequence: Synthetic peptide"
GYTFSDY

SEQ ID NO: 235 - protein, 8 aa, Artificial Sequence
  source: /note="Description of Artificial Sequence: Synthetic peptide"
GYTFSDYN

SEQ ID NO: 236 - protein, 17 aa, Artificial Sequence
  source: /note="Description of Artificial Sequence: Synthetic peptide"
QINPYNHLIFFNQKFQG

SEQ ID NO: 237 - protein, 17 aa, Artificial Sequence
  source: /note="Description of Artificial Sequence: Synthetic peptide"
QINPNNGLIFFNQKFQG

SEQ ID NO: 238 - protein, 17 aa, Artificial Sequence
  source: /note="Description of Artificial Sequence: Synthetic peptide"
QINPNNGLIFFNQKFKG

SEQ ID NO: 239 - protein, 17 aa, Artificial Sequence
  source: /note="Description of Artificial Sequence: Synthetic peptide"
QINPYNHLIFFNQKFKG

SEQ ID NO: 240 - protein, 6 aa, Artificial Sequence
  source: /note="Description of Artificial Sequence: Synthetic peptide"
NPYNHL

SEQ ID NO: 241 - protein, 6 aa, Artificial Sequence
  source: /note="Description of Artificial Sequence: Synthetic peptide"
NPNNGL

SEQ ID NO: 242 - protein, 8 aa, Artificial Sequence
  source: /note="Description of Artificial Sequence: Synthetic peptide"
INPYNHLI

SEQ ID NO: 243 - protein, 8 aa, Artificial Sequence
  source: /note="Description of Artificial Sequence: Synthetic peptide"
INPNNGLI

SEQ ID NO: 244 - protein, 9 aa, Artificial Sequence
  source: /note="Description of Artificial Sequence: Synthetic peptide"
QHFWSDPYT

SEQ ID NO: 245 - DNA, 360 bp, Artificial Sequence
  source: /note="Description of Artificial Sequence: Synthetic polynucleotide"
caggtccagcttgtgcaatcgggagcggaagtgaagaaaccgggagcgtcggtaaaagtctcgtgcaaagcgtcggggtatacgtttacggactataacatggactgggtgcgccaagcgcctggacagagccttgaatggatggggcagattaatccgtacaatcacctgatcttctttaatcagaaattccagggaagggtaacgctgacgacagacacgtcaacatcgacggcctatatggaattgcggtcgttgcgatcagatgatacggcggtctactattgtgcgagggaggcgattacgacggtgggagcgatggattattggggacaggggacgttggtaacggtatcgtcg

SEQ ID NO: 246 - protein, 120 aa, Artificial Sequence
  source: /note="Description of Artificial Sequence: Synthetic polypeptide"
QVQLVQSGAEVKKPGASVKVSCKASGYTFTDYNMDWVRQAPGQSLEWMGQINPYNHLIFFNQKFQGRVTLTTDTSTSTAYMELRSLRSDDTAVYYCAREAITTVGAMDYWGQGTLVTVSS

SEQ ID NO: 247 - DNA, 360 bp, Artificial Sequence
  source: /note="Description of Artificial Sequence: Synthetic polynucleotide"
caggtccagcttgtgcaatcgggagcggaagtgaagaaaccgggagcgtcggtaaaagtctcgtgcaaagcgtcggggtatacgtttacggactataacatggactgggtgcgccaagcgcctggacagagccttgaatggatggggcagattaatccgaataatggactgatcttctttaatcagaaattccagggaagggtaacgctgacgacagacacgtcaacatcgacggcctatatggaattgcggtcgttgcgatcagatgatacggcggtctactattgtgcgagggaggcgattacgacggtgggagcgatggattattggggacaggggacgttggtaacggtatcgtcg

SEQ ID NO: 248 - protein, 120 aa, Artificial Sequence
  source: /note="Description of Artificial Sequence: Synthetic polypeptide"
QVQLVQSGAEVKKPGASVKVSCKASGYTFTDYNMDWVRQAPGQSLEWMGQINPNNGLIFFNQKFQGRVTLTTDTSTSTAYMELRSLRSDDTAVYYCAREAITTVGAMDYWGQGTLVTVSS

SEQ ID NO: 249 - DNA, 360 bp, Artificial Sequence
  source: /note="Description of Artificial Sequence: Synthetic polynucleotide"
caagtacagcttgtacagtcgggagcggaagtcaagaaaccgggatcgtcggtcaaagtgtcgtgtaaagcgtcgggatatacgtttagcgactataacatggattgggtgcgacaagcgcctgggcagggacttgaatggatgggtcagatcaatccgaataatgggctgatctttttcaatcagaagtttaaagggagggtaacgctgacggcggataaaagcacgtcaacggcgtatatggagttgtcgtcgttgcggtcggaggacacggcggtctattactgcgcgagggaagcgattacgacggtgggagcgatggattattgggggcagggaacgcttgtaacggtgtcatcg

SEQ ID NO: 250 - protein, 120 aa, Artificial Sequence
  source: /note="Description of Artificial Sequence: Synthetic polypeptide"
QVQLVQSGAEVKKPGSSVKVSCKASGYTFSDYNMDWVRQAPGQGLEWMGQINPNNGLIFFNQKFKGRVTLTADKSTSTAYMELSSLRSEDTAVYYCAREAITTVGAMDYWGQGTLVTVSS

SEQ ID NO: 251 - DNA, 360 bp, Artificial Sequence
  source: /note="Description of Artificial Sequence: Synthetic polynucleotide"
caagtacagcttgtacagtcgggagcggaagtcaagaaaccgggatcgtcggtcaaagtgtcgtgtaaagcgtcgggatatacgtttagcgactataacatggattgggtgcgacaagcgcctgggcagggacttgaatggatgggtcagatcaatccgtacaatcacctgatctttttcaatcagaagtttaaagggagggtaacgctgacggcggataaaagcacgtcaacggcgtatatggagttgtcgtcgttgcggtcggaggacacggcggtctattactgcgcgagggaagcgattacgacggtgggagcgatggattattgggggcagggaacgcttgtaacggtgtcatcg

SEQ ID NO: 252 - protein, 120 aa, Artificial Sequence
  source: /note="Description of Artificial Sequence: Synthetic polypeptide"
QVQLVQSGAEVKKPGSSVKVSCKASGYTFSDYNMDWVRQAPGQGLEWMGQINPYNHLIFFNQKFKGRVTLTADKSTSTAYMELSSLRSEDTAVYYCAREAITTVGAMDYWGQGTLVTVSS

SEQ ID NO: 253 - DNA, 321 bp, Artificial Sequence
  source: /note="Description of Artificial Sequence: Synthetic polynucleotide"
gacatccaaatgacccagtcgccgtcgtcgctttcagcgtcggtaggggatcgggtcacaattacgtgccgaacgtcagagaatttgcataactacctcgcgtggtatcagcagaagcccgggaagtcaccgaaactccttatctacgatgcgaaaacgctggcggatggagtgccgtcgagattctcgggaagcggatccggtacggactatacgcttacgatctcatcgctccagcccgaggactttgcgacgtactattgtcagcatttttggtcggacccctacacatttgggcaggggaccaagttggaaatcaag

SEQ ID NO: 254 - protein, 107 aa, Artificial Sequence
  source: /note="Description of Artificial Sequence: Synthetic polypeptide"
DIQMTQSPSSLSASVGDRVTITCRTSENLHNYLAWYQQKPGKSPKLLIYDAKTLADGVPSRFSGSGSGTDYTLTISSLQPEDFATYYCQHFWSDPYTFGQGTKLEIK

SEQ ID NO: 255 - DNA, 1350 bp, Artificial Sequence
  source: /note="Description of Artificial Sequence: Synthetic polynucleotide"
caggtccagcttgtgcaatcgggagcggaagtgaagaaaccgggagcgtcggtaaaagtctcgtgcaaagcgtcggggtatacgtttacggactataacatggactgggtgcgccaagcgcctggacagagccttgaatggatggggcagattaatccgtacaatcacctgatcttctttaatcagaaattccagggaagggtaacgctgacgacagacacgtcaacatcgacggcctatatggaattgcggtcgttgcgatcagatgatacggcggtctactattgtgcgagggaggcgattacgacggtgggagcgatggattattggggacaggggacgttggtaacggtatcgtcggcctcaacaaaaggaccaagtgtgttcccactcgcccctagcagcaagagtacatccgggggcactgcagcactcggctgcctcgtcaaggattattttccagagccagtaaccgtgagctggaacagtggagcactcacttctggtgtccatacttttcctgctgtcctgcaaagctctggcctgtactcactcagctccgtcgtgaccgtgccatcttcatctctgggcactcagacctacatctgtaatgtaaaccacaagcctagcaatactaaggtcgataagcgggtggaacccaagagctgcgacaagactcacacttgtcccccatgccctgcccctgaacttctgggcggtcccagcgtctttttgttcccaccaaagcctaaagatactctgatgataagtagaacacccgaggtgacatgtgttgttgtagacgtttcccacgaggacccagaggttaagttcaactggtacgttgatggagtcgaagtacataatgctaagaccaagcctagagaggagcagtataatagtacataccgtgtagtcagtgttctcacagtgctgcaccaagactggctcaacggcaaagaatacaaatgcaaagtgtccaacaaagcactcccagcccctatcgagaagactattagtaaggcaaaggggcagcctcgtgaaccacaggtgtacactctgccacccagtagagaggaaatgacaaagaaccaagtctcattgacctgcctggtgaaaggcttctaccccagcgacatcgccgttgagtgggagagtaacggtcagcctgagaacaattacaagacaacccccccagtgctggatagtgacgggtctttctttctgtacagtaagctgactgtggacaagtcccgctggcagcagggtaacgtcttcagctgttccgtgatgcacgaggcattgcacaaccactacacccagaagtcactgagcctgagcccagggaag

SEQ ID NO: 256 - protein, 450 aa, Artificial Sequence
  source: /note="Description of Artificial Sequence: Synthetic polypeptide"
QVQLVQSGAEVKKPGASVKVSCKASGYTFTDYNMDWVRQAPGQSLEWMGQINPYNHLIFFNQKFQGRVTLTTDTSTSTAYMELRSLRSDDTAVYYCAREAITTVGAMDYWGQGTLVTVSSASTKGPSVFPLAPSSKSTSGGTAALGCLVKDYFPEPVTVSWNSGALTSGVHTFPAVLQSSGLYSLSSVVTVPSSSLGTQTYICNVNHKPSNTKVDKRVEPKSCDKTHTCPPCPAPELLGGPSVFLFPPKPKDTLMISRTPEVTCVVVDVSHEDPEVKFNWYVDGVEVHNAKTKPREEQYNSTYRVVSVLTVLHQDWLNGKEYKCKVSNKALPAPIEKTISKAKGQPREPQVYTLPPSREEMTKNQVSLTCLVKGFYPSDIAVEWESNGQPENNYKTTPPVLDSDGSFFLYSKLTVDKSRWQQGNVFSCSVMHEALHNHYTQKSLSLSPGK

SEQ ID NO: 257 - DNA, 1350 bp, Artificial Sequence
  source: /note="Description of Artificial Sequence: Synthetic polynucleotide"
caggtccagcttgtgcaatcgggagcggaagtgaagaaaccgggagcgtcggtaaaagtctcgtgcaaagcgtcggggtatacgtttacggactataacatggactgggtgcgccaagcgcctggacagagccttgaatggatggggcagattaatccgaataatggactgatcttctttaatcagaaattccagggaagggtaacgctgacgacagacacgtcaacatcgacggcctatatggaattgcggtcgttgcgatcagatgatacggcggtctactattgtgcgagggaggcgattacgacggtgggagcgatggattattggggacaggggacgttggtaacggtatcgtcggcctcaacaaaaggaccaagtgtgttcccactcgcccctagcagcaagagtacatccgggggcactgcagcactcggctgcctcgtcaaggattattttccagagccagtaaccgtgagctggaacagtggagcactcacttctggtgtccatacttttcctgctgtcctgcaaagctctggcctgtactcactcagctccgtcgtgaccgtgccatcttcatctctgggcactcagacctacatctgtaatgtaaaccacaagcctagcaatactaaggtcgataagcgggtggaacccaagagctgcgacaagactcacacttgtcccccatgccctgcccctgaacttctgggcggtcccagcgtctttttgttcccaccaaagcctaaagatactctgatgataagtagaacacccgaggtgacatgtgttgttgtagacgtttcccacgaggacccagaggttaagttcaactggtacgttgatggagtcgaagtacataatgctaagaccaagcctagagaggagcagtataatagtacataccgtgtagtcagtgttctcacagtgctgcaccaagactggctcaacggcaaagaatacaaatgcaaagtgtccaacaaagcactcccagcccctatcgagaagactattagtaaggcaaaggggcagcctcgtgaaccacaggtgtacactctgccacccagtagagaggaaatgacaaagaaccaagtctcattgacctgcctggtgaaaggcttctaccccagcgacatcgccgttgagtgggagagtaacggtcagcctgagaacaattacaagacaacccccccagtgctggatagtgacgggtctttctttctgtacagtaagctgactgtggacaagtcccgctggcagcagggtaacgtcttcagctgttccgtgatgcacgaggcattgcacaaccactacacccagaagtcactgagcctgagcccagggaag

SEQ ID NO: 258 - protein, 450 aa, Artificial Sequence
  source: /note="Description of Artificial Sequence: Synthetic polypeptide"
QVQLVQSGAEVKKPGASVKVSCKASGYTFTDYNMDWVRQAPGQSLEWMGQINPNNGLIFFNQKFQGRVTLTTDTSTSTAYMELRSLRSDDTAVYYCAREAITTVGAMDYWGQGTLVTVSSASTKGPSVFPLAPSSKSTSGGTAALGCLVKDYFPEPVTVSWNSGALTSGVHTFPAVLQSSGLYSLSSVVTVPSSSLGTQTYICNVNHKPSNTKVDKRVEPKSCDKTHTCPPCPAPELLGGPSVFLFPPKPKDTLMISRTPEVTCVVVDVSHEDPEVKFNWYVDGVEVHNAKTKPREEQYNSTYRVVSVLTVLHQDWLNGKEYKCKVSNKALPAPIEKTISKAKGQPREPQVYTLPPSREEMTKNQVSLTCLVKGFYPSDIAVEWESNGQPENNYKTTPPVLDSDGSFFLYSKLTVDKSRWQQGNVFSCSVMHEALHNHYTQKSLSLSPGK

SEQ ID NO: 259 - DNA, 1350 bp, Artificial Sequence
  source: /note="Description of Artificial Sequence: Synthetic polynucleotide"
caagtacagcttgtacagtcgggagcggaagtcaagaaaccgggatcgtcggtcaaagtgtcgtgtaaagcgtcgggatatacgtttagcgactataacatggattgggtgcgacaagcgcctgggcagggacttgaatggatgggtcagatcaatccgaataatgggctgatctttttcaatcagaagtttaaagggagggtaacgctgacggcggataaaagcacgtcaacggcgtatatggagttgtcgtcgttgcggtcggaggacacggcggtctattactgcgcgagggaagcgattacgacggtgggagcgatggattattgggggcagggaacgcttgtaacggtgtcatcggcctcaacaaaaggaccaagtgtgttcccactcgcccctagcagcaagagtacatccgggggcactgcagcactcggctgcctcgtcaaggattattttccagagccagtaaccgtgagctggaacagtggagcactcacttctggtgtccatacttttcctgctgtcctgcaaagctctggcctgtactcactcagctccgtcgtgaccgtgccatcttcatctctgggcactcagacctacatctgtaatgtaaaccacaagcctagcaatactaaggtcgataagcgggtggaacccaagagctgcgacaagactcacacttgtcccccatgccctgcccctgaacttctgggcggtcccagcgtctttttgttcccaccaaagcctaaagatactctgatgataagtagaacacccgaggtgacatgtgttgttgtagacgtttcccacgaggacccagaggttaagttcaactggtacgttgatggagtcgaagtacataatgctaagaccaagcctagagaggagcagtataatagtacataccgtgtagtcagtgttctcacagtgctgcaccaagactggctcaacggcaaagaatacaaatgcaaagtgtccaacaaagcactcccagcccctatcgagaagactattagtaaggcaaaggggcagcctcgtgaaccacaggtgtacactctgccacccagtagagaggaaatgacaaagaaccaagtctcattgacctgcctggtgaaaggcttctaccccagcgacatcgccgttgagtgggagagtaacggtcagcctgagaacaattacaagacaacccccccagtgctggatagtgacgggtctttctttctgtacagtaagctgactgtggacaagtcccgctggcagcagggtaacgtcttcagctgttccgtgatgcacgaggcattgcacaaccactacacccagaagtcactgagcctgagcccagggaag

SEQ ID NO: 260 - protein, 450 aa, Artificial Sequence
  source: /note="Description of Artificial Sequence: Synthetic polypeptide"
QVQLVQSGAEVKKPGSSVKVSCKASGYTFSDYNMDWVRQAPGQGLEWMGQINPNNGLIFFNQKFKGRVTLTADKSTSTAYMELSSLRSEDTAVYYCAREAITTVGAMDYWGQGTLVTVSSASTKGPSVFPLAPSSKSTSGGTAALGCLVKDYFPEPVTVSWNSGALTSGVHTFPAVLQSSGLYSLSSVVTVPSSSLGTQTYICNVNHKPSNTKVDKRVEPKSCDKTHTCPPCPAPELLGGPSVFLFPPKPKDTLMISRTPEVTCVVVDVSHEDPEVKFNWYVDGVEVHNAKTKPREEQYNSTYRVVSVLTVLHQDWLNGKEYKCKVSNKALPAPIEKTISKAKGQPREPQVYTLPPSREEMTKNQVSLTCLVKGFYPSDIAVEWESNGQPENNYKTTPPVLDSDGSFFLYSKLTVDKSRWQQGNVFSCSVMHEALHNHYTQKSLSLSPGK

SEQ ID NO: 261 - DNA, 1350 bp, Artificial Sequence
  source: /note="Description of Artificial Sequence: Synthetic polynucleotide"
caagtacagcttgtacagtcgggagcggaagtcaagaaaccgggatcgtcggtcaaagtgtcgtgtaaagcgtcgggatatacgtttagcgactataacatggattgggtgcgacaagcgcctgggcagggacttgaatggatgggtcagatcaatccgtacaatcacctgatctttttcaatcagaagtttaaagggagggtaacgctgacggcggataaaagcacgtcaacggcgtatatggagttgtcgtcgttgcggtcggaggacacggcggtctattactgcgcgagggaagcgattacgacggtgggagcgatggattattgggggcagggaacgcttgtaacggtgtcatcggcctcaacaaaaggaccaagtgtgttcccactcgcccctagcagcaagagtacatccgggggcactgcagcactcggctgcctcgtcaaggattattttccagagccagtaaccgtgagctggaacagtggagcactcacttctggtgtccatacttttcctgctgtcctgcaaagctctggcctgtactcactcagctccgtcgtgaccgtgccatcttcatctctgggcactcagacctacatctgtaatgtaaaccacaagcctagcaatactaaggtcgataagcgggtggaacccaagagctgcgacaagactcacacttgtcccccatgccctgcccctgaacttctgggcggtcccagcgtctttttgttcccaccaaagcctaaagatactctgatgataagtagaacacccgaggtgacatgtgttgttgtagacgtttcccacgaggacccagaggttaagttcaactggtacgttgatggagtcgaagtacataatgctaagaccaagcctagagaggagcagtataatagtacataccgtgtagtcagtgttctcacagtgctgcaccaagactggctcaacggcaaagaatacaaatgcaaagtgtccaacaaagcactcccagcccctatcgagaagactattagtaaggcaaaggggcagcctcgtgaaccacaggtgtacactctgccacccagtagagaggaaatgacaaagaaccaagtctcattgacctgcctggtgaaaggcttctaccccagcgacatcgccgttgagtgggagagtaacggtcagcctgagaacaattacaagacaacccccccagtgctggatagtgacgggtctttctttctgtacagtaagctgactgtggacaagtcccgctggcagcagggtaacgtcttcagctgttccgtgatgcacgaggcattgcacaaccactacacccagaagtcactgagcctgagcccagggaag

SEQ ID NO: 262 - protein, 450 aa, Artificial Sequence
  source: /note="Description of Artificial Sequence: Synthetic polypeptide"
QVQLVQSGAEVKKPGSSVKVSCKASGYTFSDYNMDWVRQAPGQGLEWMGQINPYNHLIFFNQKFKGRVTLTADKSTSTAYMELSSLRSEDTAVYYCAREAITTVGAMDYWGQGTLVTVSSASTKGPSVFPLAPSSKSTSGGTAALGCLVKDYFPEPVTVSWNSGALTSGVHTFPAVLQSSGLYSLSSVVTVPSSSLGTQTYICNVNHKPSNTKVDKRVEPKSCDKTHTCPPCPAPELLGGPSVFLFPPKPKDTLMISRTPEVTCVVVDVSHEDPEVKFNWYVDGVEVHNAKTKPREEQYNSTYRVVSVLTVLHQDWLNGKEYKCKVSNKALPAPIEKTISKAKGQPREPQVYTLPPSREEMTKNQVSLTCLVKGFYPSDIAVEWESNGQPENNYKTTPPVLDSDGSFFLYSKLTVDKSRWQQGNVFSCSVMHEALHNHYTQKSLSLSPGK

SEQ ID NO: 263 - DNA, 642 bp, Artificial Sequence
  source: /note="Description of Artificial Sequence: Synthetic polynucleotide"
gacatccaaatgacccagtcgccgtcgtcgctttcagcgtcggtaggggatcgggtcacaattacgtgccgaacgtcagagaatttgcataactacctcgcgtggtatcagcagaagcccgggaagtcaccgaaactccttatctacgatgcgaaaacgctggcggatggagtgccgtcgagattctcgggaagcggatccggtacggactatacgcttacgatctcatcgctccagcccgaggactttgcgacgtactattgtcagcatttttggtcggacccctacacatttgggcaggggaccaagttggaaatcaagcgcacagttgctgcccccagcgtgttcattttcccacctagcgatgagcagctgaaaagcggtactgcctctgtcgtatgcttgctcaacaacttttacccacgtgaggctaaggtgcagtggaaagtggataatgcacttcaatctggaaacagtcaagagtccgtgacagaacaggacagcaaagactcaacttattcactctcttccaccctgactctgtccaaggcagactatgaaaaacacaaggtatacgcctgcgaggttacacaccagggtttgtctagtcctgtcaccaagtccttcaataggggcgaatgt

SEQ ID NO: 264 - protein, 214 aa, Artificial Sequence
  source: /note="Description of Artificial Sequence: Synthetic polypeptide"
DIQMTQSPSSLSASVGDRVTITCRTSENLHNYLAWYQQKPGKSPKLLIYDAKTLADGVPSRFSGSGSGTDYTLTISSLQPEDFATYYCQHFWSDPYTFGQGTKLEIKRTVAAPSVFIFPPSDEQLKSGTASVVCLLNNFYPREAKVQWKVDNALQSGNSQESVTEQDSKDSTYSLSSTLTLSKADYEKHKVYACEVTHQGLSSPVTKSFNRGEC

SEQ ID NO: 265 - protein, 4 aa, Artificial Sequence
  source: /note="Description of Artificial Sequence: Synthetic peptide"
GGGG

SEQ ID NO: 266 - protein, 6 aa, Artificial Sequence
  source: /note="Description of Artificial Sequence: Synthetic 6xHis tag"
HHHHHH